European Patent Application EP 4 455 290 A1, published October 30, 2024. Title: A fusion protein of an anti-transferrin receptor antibody and a physiologically active protein for safe gene therapy. Applicant: JCR Pharmaceuticals Co., Ltd. The sequence listing filed with the application follows.

SEQUENCE LISTING (64 sequences)

SEQ ID NO: 1 - protein, 5 aa, synthetic construct
GGGGS

SEQ ID NO: 2 - protein, 6 aa, synthetic construct
GGGGGS

SEQ ID NO: 3 - protein, 5 aa, synthetic construct
SGGGG

SEQ ID NO: 4 - protein, 15 aa, synthetic construct
GGGGSGGGGSGGGGS

SEQ ID NO: 5 - DNA, 145 bp, Adeno-associated virus serotype 2
  source 1..145: mol_type = genomic DNA
ttggccactccctctctgcgcgctcgctcgctcactgaggccgggcgaccaaaggtcgcccgacgcccgggctttgcccgggcggcctcagtgagcgagcgagcgcgcagagagggagtggccaactccatcactaggggttcct

SEQ ID NO: 6 - DNA, 145 bp, Adeno-associated virus serotype 2
  source 1..145: mol_type = genomic DNA
aggaacccctagtgatggagttggccactccctctctgcgcgctcgctcgctcactgaggccgggcgaccaaaggtcgcccgacgcccgggctttgcccgggcggcctcagtgagcgagcgagcgcgcagagagggagtggccaa

SEQ ID NO: 7 - DNA, 141 bp, synthetic construct
  source 1..141: mol_type = other DNA
cctgcaggcagctgcgcgctcgctcgctcactgaggccgcccgggcaaagcccgggcgtcgggcgacctttggtcgcccggcctcagtgagcgagcgagcgcgcagagagggagtggccaactccatcactaggggttcct

SEQ ID NO: 8 - DNA, 141 bp, synthetic construct
  source 1..141: mol_type = other DNA
aggaacccctagtgatggagttggccactccctctctgcgcgctcgctcgctcactgaggccgggcgaccaaaggtcgcccgacgcccgggctttgcccgggcggcctcagtgagcgagcgagcgcgcagctgcctgcagg

SEQ ID NO: 9 - DNA, 559 bp, Mus musculus
  source 1..559: mol_type = genomic DNA
agatcattttgatggcagagttcagtttaccgggtcacattgtacctgggaagattcaaggatttatggaaaaagtcaacaacaggagtcagagcagccggaaaagcatggactctgtacttaggactgcgctttgagcaatggcacagcaagctataaccctgtttgcagtcagcacacaaactgtggttcaaagctccactttatctcttcttgtggaattcagatatcagatcagttttgctcaaatgggagacaaagagattaagctcttatgtaaaatttgctgttttacataactttaatgaatggacaaagtcttgtgcatgggggtgggggtggggttagaggggaacagctccagatggcaaacatacgcaagggatttagtcaaacaactttttggcaaagatggtatgattttgtaatggggtaggaaccaatgaaatgcgaggtaagtatggttaataatctacagttattggttaaagaagtatattagagcgagtctttctgcacacagatcaccttcctatcaaccccactagcctctggcaaa

SEQ ID NO: 10 - DNA, 225 bp, Gallus gallus
  source 1..225: mol_type = genomic DNA
ggagtcgctgcgttgccttcgccccgtgccccgctccgcgccgcctcgcgccgcccgccccggctctgactgaccgcgttactcccacaggtgagcgggcgggacggcccttctcctccgggctgtaattagcaagaggtaagggtttaagggatggttggttggtggggtattaatgtttaattacctggagcacctgcctgaaatcactttttttcaggttgg

SEQ ID NO: 11 - DNA, 593 bp, mouse encephalomyocarditis virus
  source 1..593: mol_type = genomic DNA
cccccccccctctccctcccccccccctaacgttactggccgaagccgcttggaataaggccggtgtgcgtttgtctatatgttattttccaccatattgccgtcttttggcaatgtgagggcccggaaacctggccctgtcttcttgacgagcattcctaggggtctttcccctctcgccaaaggaatgcaaggtctgttgaatgtcgtgaaggaagcagttcctctggaagcttcttgaagacaaacaacgtctgtagcgaccctttgcaggcagcggaaccccccacctggcgacaggtgcctctgcggccaaaagccacgtgtataagatacacctgcaaaggcggcacaaccccagtgccacgttgtgagttggatagttgtggaaagagtcaaatggctctcctcaagcgtattcaacaaggggctgaaggatgcccagaaggtaccccattgtatgggatctgatctggggcctcggtgcacatgctttacatgtgtttagtcgaggttaaaaaaacgtctaggccccccgaaccacggggacgtggttttcctttgaaaaacacgatgataatatggccacaacc

SEQ ID NO: 12 - protein, 760 aa, Homo sapiens
MMDQARSAFSNLFGGEPLSYTRFSLARQVDGDNSHVEMKLAVDEEENADNNTKANVTKPKRCSGSICYGTIAVIVFFLIGFMIGYLGYCKGVEPKTECERLAGTESPVREEPGEDFPAARRLYWDDLKRKLSEKLDSTDFTGTIKLLNENSYVPREAGSQKDENLALYVENQFREFKLSKVWRDQHFVKIQVKDSAQNSVIIVDKNGRLVYLVENPGGYVAYSKAATVTGKLVHANFGTKKDFEDLYTPVNGSIVIVRAGKITFAEKVANAESLNAIGVLIYMDQTKFPIVNAELSFFGHAHLGTGDPYTPGFPSFNHTQFPPSRSSGLPNIPVQTISRAAAEKLFGNMEGDCPSDWKTDSTCRMVTSESKNVKLTVSNVLKEIKILNIFGVIKGFVEPDHYVVVGAQRDAWGPGAAKSGVGTALLLKLAQMFSDMVLKDGFQPSRSIIFASWSAGDFGSVGATEWLEGYLSSLHLKAFTYINLDKAVLGTSNFKVSASPLLYTLIEKTMQNVKHPVTGQFLYQDSNWASKVEKLTLDNAAFPFLAYSGIPAVSFCFCEDTDYPYLGTTMDTYKELIERIPELNKVARAAAEVAGQFVIKLTHDVELNLDYERYNSQLLSFVRDLNQYRADIKEMGLSLQWLYSARGDFFRATSRLTTDFGNAEKTDRFVMKKLNDRVMRVEYHFLSPYVSPKESPFRHVFWGSGSHTLPALLENLKLRKQNNGAFNETLFRNQLALATWTIQGAANALSGDVWDIDNEF

SEQ ID NO: 13 - protein, 226 aa, synthetic construct
EVQLVQSGAEVKKPGESLKISCKGSGYSFMNYWLGWVRQMPGKGLEWMGDIYPGGDYPTYSEKFKVQVTISADKSISTAYLQLSSLKASDTAMYYCARSGNYDEVAYWGQGTLVTVSSASTKGPSVFPLAPSSKSTSGGTAALGCLVKDYFPEPVTVSWNSGALTSGVHTFPAVLQSSGLYSLSSVVTVPSSSLGTQTYICNVNHKPSNTKVDKKVEPKSCDKTHT

SEQ ID NO: 14 - protein, 525 aa, Homo sapiens
SETQANSTTDALNVLLIIVDDLRPSLGCYGDKLVRSPNIDQLASHSLLFQNAFAQQAVCAPSRVSFLTGRRPDTTRLYDFNSYWRVHAGNFSTIPQYFKENGYVTMSVGKVFHPGISSNHTDDSPYSWSFPPYHPSSEKYENTKTCRGPDGELHANLLCPVDVLDVPEGTLPDKQSTEQAIQLLEKMKTSASPFFLAVGYHKPHIPFRYPKEFQKLYPLENITLAPDPEVPDGLPPVAYNPWMDIRQREDVQALNISVPYGPIPVDFQRKIRQSYFASVSYLDTQVGRLLSALDDLQLANSTIIAFTSDHGWALGEHGEWAKYSNFDVATHVPLIFYVPGRTASLPEAGEKLFPYLDPFDSASQLMEPGRQSMDLVELVSLFPTLAGLAGLQVPPRCPVPSFHVELCREGKNLLKHFRFRDLEEDPYLPGNPRELIAYSQYPRPSDIPQWNSDKPSLKDIKIMGYSIRTIDYRYTVWVGFNPDEFLANFSDIHAGELYFVDSDPLQDHNMYNDSQGGDLFQLLMP

SEQ ID NO: 15 - protein, 219 aa, synthetic construct
DIVMTQTPLSLSVTPGQPASISCRSSQSLVHSNGNTYLHWYLQKPGQSPQLLIYKVSNRFSGVPDRFSGSGSGTDFTLKISRVEAEDVGVYYCSQSTHVPWTFGQGTKVEIKRTVAAPSVFIFPPSDEQLKSGTASVVCLLNNFYPREAKVQWKVDNALQSGNSQESVTEQDSKDSTYSLSSTLTLSKADYEKHKVYACEVTHQGLSSPVTKSFNRGEC

SEQ ID NO: 16 - protein, 226 aa, synthetic construct; identical to SEQ ID NO: 13

SEQ ID NO: 17 - DNA, 208 bp, Bos taurus
  source 1..208: mol_type = genomic DNA
ctgtgccttctagttgccagccatctgttgtttgcccctcccccgtgccttccttgaccctggaaggtgccactcccactgtcctttcctaataaaatgaggaaattgcatcgcattgtctgagtaggtgtcattctattctggggggtggggtggggcaggacagcaagggggaggattgggaagacaatagcaggcatgctgggga

SEQ ID NO: 18 - DNA, 3465 bp, synthetic construct
  source 1..3465: mol_type = other DNA
atcgatatcaagcttagatcattttgatggcagagttcagtttaccgggtcacattgtacctgggaagattcaaggatttatggaaaaagtcaacaacaggagtcagagcagccggaaaagcatggactctgtacttaggactgcgctttgagcaatggcacagcaagctataaccctgtttgcagtcagcacacaaactgtggttcaaagctccactttatctcttcttgtggaattcagatatcagatcagttttgctcaaatgggagacaaagagattaagctcttatgtaaaatttgctgttttacataactttaatgaatggacaaagtcttgtgcatgggggtgggggtggggttagaggggaacagctccagatggcaaacatacgcaagggatttagtcaaacaactttttggcaaagatggtatgattttgtaatggggtaggaaccaatgaaatgcgaggtaagtatggttaataatctacagttattggttaaagaagtatattagagcgagtctttctgcacacagatcaccttcctatcaaccccactagcctctggcaaaggtaccagtgtacagggagtcgctgcgttgccttcgccccgtgccccgctccgcgccgcctcgcgccgcccgccccggctctgactgaccgcgttactcccacaggtgagcgggcgggacggcccttctcctccgggctgtaattagcaagaggtaagggtttaagggatggttggttggtggggtattaatgtttaattacctggagcacctgcctgaaatcactttttttcaggttggacgcgtgccgccaccatgggctggagctgcattattctgtttctggtggcgaccgcgaccggcgtgcatagcgaggtgcagctggtggagagcggcggcggcctggtgcagcccggcaacagcctgaccctgagctgcgtggccagcggcttcaccttcagcaactacggcatgcactggatcaggcaggcccccaagaagggcctggagtggatcgccatgatctactacgacagcagcaagatgaactacgccgacaccgtgaagggccgcttcaccatcagccgcgacaacagcaagaacaccctgtacctggagatgaacagcctgcgcagcgaggacaccgccatgtactactgcgccgtgcccaccagccactacgtggtggacgtgtggggacaaggcgtgagcgtgaccgtgagcagcggtggcggagggtctggcggaggaggttccgggggcggtggaagcgacatccagatgacccagagccccgccagtctgagcgccagcctggaggagatcgtgaccatcacctgccaggcaagccaagacatcggcaactggctggcctggtaccagcagaagcccggcaagagcccccagctgctgatctacggcgccaccagcctggccgacggcgtgcccagccgcttcagcggcagccgcagcggcacccagttcagcctgaagatcagccgcgtgcaggtggaggacatcggcatctactactgcctgcaggcctacaacaccccctggaccttcggcggcggcaccaagctggagctgaagcgcggtggcggagggtctggaggtggcggatcaggcggaggaggatcttccgaaacgcaggccaactcgaccacagatgctctgaacgttcttctcatcatcgtggatgacctgcgcccctccctgggctgttatggggataagctggtgaggtccccaaatattgaccaactggcatcccacagcctcctcttccagaatgcctttgcgcagcaagcagtgtgcgccccgagccgcgtttctttcctcactggcaggagacctgacaccacccgcctgtacgacttcaactcctactggagggtgcacgctggaaacttctccaccatcccccagtacttcaaggagaatggctatgtgaccatgtcggtgggaaaagtctttcaccctgggatatcttctaaccataccgatgattctccgtatagctggtcttttccaccttatcatccttcctctgagaagtatgaaaacactaagacatgtcgagggccagatggagaactccatgccaacctgctttgccctgtggatgtgctggatgttcccgagggcaccttgcctgacaaacagagcactgagcaagccatacagttgttggaaaagatgaaaacgtcagccagtcctttcttcctggccgttgggtatcataagccacacatccccttcagataccccaaggaatttcagaagttgtatcccttggagaacatcaccctggcccccgatcccgaggtccctgatggcctaccccctgtggcctacaacccctggatggacatcaggcaacgggaagacgtccaagccttaaacatcagtgtgccgtatggtccaattcctgtggactttcagcggaaaatccgccagagctactttgcctctgtgtcatatttggatacacaggtcggccgcctcttgagtgctttggacgatcttcagctggccaacagcaccatcattgcatttacctcggatcatgggtgggctctaggtgaacatggagaatgggccaaatacagcaattttgatgttgctacccatgttcccctgatattctatgttcctggaaggacggcttcacttccggaggcaggcgagaagcttttcccttacctcgacccttttgattccgcctcacagttgatggagccaggcaggcaatccatggaccttgtggaacttgtgtctctttttcccacgctggctggacttgcaggactgcaggttccacctcgctgccccgttccttcatttcacgttgagctgtgcagagaaggcaagaaccttctgaagcattttcgattccgtgacttggaagaagatccgtacctccctggtaatccccgtgaactgattgcctatagccagtatccccggccttcagacatccctcagtggaattctgacaagccgagtttaaaagatataaagatcatgggctattccatacgcaccatagactataggtatactgtgtgggttggcttcaatcctgatgaatttctagctaacttttctgacatccatgcaggggaactgtattttgtggattctgacccattgcaggatcacaatatgtataatgattcccaaggtggagaccttttccagttgttgatgccttaataagcggccgcatttaaatctgtgccttctagttgccagccatctgttgtttgcccctcccccgtgccttccttgaccctggaaggtgccactcccactgtcctttcctaataaaatgaggaaattgcatcgcattgtctgagtaggtgtcattctattctggggggtggggtggggcaggacagcaagggggaggattgggaagacaatagcaggcatgctggggaagatct

SEQ ID NO: 19 - protein, 781 aa, synthetic construct
EVQLVESGGGLVQPGNSLTLSCVASGFTFSNYGMHWIRQAPKKGLEWIAMIYYDSSKMNYADTVKGRFTISRDNSKNTLYLEMNSLRSEDTAMYYCAVPTSHYVVDVWGQGVSVTVSSGGGGSGGGGSGGGGSDIQMTQSPASLSASLEEIVTITCQASQDIGNWLAWYQQKPGKSPQLLIYGATSLADGVPSRFSGSRSGTQFSLKISRVQVEDIGIYYCLQAYNTPWTFGGGTKLELKRGGGGSGGGGSGGGGSSETQANSTTDALNVLLIIVDDLRPSLGCYGDKLVRSPNIDQLASHSLLFQNAFAQQAVCAPSRVSFLTGRRPDTTRLYDFNSYWRVHAGNFSTIPQYFKENGYVTMSVGKVFHPGISSNHTDDSPYSWSFPPYHPSSEKYENTKTCRGPDGELHANLLCPVDVLDVPEGTLPDKQSTEQAIQLLEKMKTSASPFFLAVGYHKPHIPFRYPKEFQKLYPLENITLAPDPEVPDGLPPVAYNPWMDIRQREDVQALNISVPYGPIPVDFQRKIRQSYFASVSYLDTQVGRLLSALDDLQLANSTIIAFTSDHGWALGEHGEWAKYSNFDVATHVPLIFYVPGRTASLPEAGEKLFPYLDPFDSASQLMEPGRQSMDLVELVSLFPTLAGLAGLQVPPRCPVPSFHVELCREGKNLLKHFRFRDLEEDPYLPGNPRELIAYSQYPRPSDIPQWNSDKPSLKDIKIMGYSIRTIDYRYTVWVGFNPDEFLANFSDIHAGELYFVDSDPLQDHNMYNDSQGGDLFQLLMP

SEQ ID NO: 20 - DNA, 2403 bp, synthetic construct
  source 1..2403: mol_type = other DNA
atgggctggagctgcattattctgtttctggtggcgaccgcgaccggcgtgcatagcgaggtgcagctggtggagagcggcggcggcctggtgcagcccggcaacagcctgaccctgagctgcgtggccagcggcttcaccttcagcaactacggcatgcactggatcaggcaggcccccaagaagggcctggagtggatcgccatgatctactacgacagcagcaagatgaactacgccgacaccgtgaagggccgcttcaccatcagccgcgacaacagcaagaacaccctgtacctggagatgaacagcctgcgcagcgaggacaccgccatgtactactgcgccgtgcccaccagccactacgtggtggacgtgtggggacaaggcgtgagcgtgaccgtgagcagcggtggcggagggtctggcggaggaggttccgggggcggtggaagcgacatccagatgacccagagccccgccagtctgagcgccagcctggaggagatcgtgaccatcacctgccaggcaagccaagacatcggcaactggctggcctggtaccagcagaagcccggcaagagcccccagctgctgatctacggcgccaccagcctggccgacggcgtgcccagccgcttcagcggcagccgcagcggcacccagttcagcctgaagatcagccgcgtgcaggtggaggacatcggcatctactactgcctgcaggcctacaacaccccctggaccttcggcggcggcaccaagctggagctgaagcgcggtggcggagggtctggaggtggcggatcaggcggaggaggatcttccgaaacgcaggccaactcgaccacagatgctctgaacgttcttctcatcatcgtggatgacctgcgcccctccctgggctgttatggggataagctggtgaggtccccaaatattgaccaactggcatcccacagcctcctcttccagaatgcctttgcgcagcaagcagtgtgcgccccgagccgcgtttctttcctcactggcaggagacctgacaccacccgcctgtacgacttcaactcctactggagggtgcacgctggaaacttctccaccatcccccagtacttcaaggagaatggctatgtgaccatgtcggtgggaaaagtctttcaccctgggatatcttctaaccataccgatgattctccgtatagctggtcttttccaccttatcatccttcctctgagaagtatgaaaacactaagacatgtcgagggccagatggagaactccatgccaacctgctttgccctgtggatgtgctggatgttcccgagggcaccttgcctgacaaacagagcactgagcaagccatacagttgttggaaaagatgaaaacgtcagccagtcctttcttcctggccgttgggtatcataagccacacatccccttcagataccccaaggaatttcagaagttgtatcccttggagaacatcaccctggcccccgatcccgaggtccctgatggcctaccccctgtggcctacaacccctggatggacatcaggcaacgggaagacgtccaagccttaaacatcagtgtgccgtatggtccaattcctgtggactttcagcggaaaatccgccagagctactttgcctctgtgtcatatttggatacacaggtcggccgcctcttgagtgctttggacgatcttcagctggccaacagcaccatcattgcatttacctcggatcatgggtgggctctaggtgaacatggagaatgggccaaatacagcaattttgatgttgctacccatgttcccctgatattctatgttcctggaaggacggcttcacttccggaggcaggcgagaagcttttcccttacctcgacccttttgattccgcctcacagttgatggagccaggcaggcaatccatggaccttgtggaacttgtgtctctttttcccacgctggctggacttgcaggactgcaggttccacctcgctgccccgttccttcatttcacgttgagctgtgcagagaaggcaagaaccttctgaagcattttcgattccgtgacttggaagaagatccgtacctccctggtaatccccgtgaactgattgcctatagccagtatccccggccttcagacatccctcagtggaattctgacaagccgagtttaaaagatataaagatcatgggctattccatacgcaccatagactataggtatactgtgtgggttggcttcaatcctgatgaatttctagctaacttttctgacatccatgcaggggaactgtattttgtggattctgacccattgcaggatcacaatatgtataatgattcccaaggtggagaccttttccagttgttgatgccttaa

SEQ ID NO: 21 - DNA, 3459 bp, synthetic construct
  source 1..3459: mol_type = other DNA
atcaagcttagatcattttgatggcagagttcagtttaccgggtcacattgtacctgggaagattcaaggatttatggaaaaagtcaacaacaggagtcagagcagccggaaaagcatggactctgtacttaggactgcgctttgagcaatggcacagcaagctataaccctgtttgcagtcagcacacaaactgtggttcaaagctccactttatctcttcttgtggaattcagatatcagatcagttttgctcaaatgggagacaaagagattaagctcttatgtaaaatttgctgttttacataactttaatgaatggacaaagtcttgtgcatgggggtgggggtggggttagaggggaacagctccagatggcaaacatacgcaagggatttagtcaaacaactttttggcaaagatggtatgattttgtaatggggtaggaaccaatgaaatgcgaggtaagtatggttaataatctacagttattggttaaagaagtatattagagcgagtctttctgcacacagatcaccttcctatcaaccccactagcctctggcaaaggtaccagtgtacagggagtcgctgcgttgccttcgccccgtgccccgctccgcgccgcctcgcgccgcccgccccggctctgactgaccgcgttactcccacaggtgagcgggcgggacggcccttctcctccgggctgtaattagcaagaggtaagggtttaagggatggttggttggtggggtattaatgtttaattacctggagcacctgcctgaaatcactttttttcaggttggacgcgtgccgccaccatgggctggagctgcattattctgtttctggtggcgaccgcgaccggcgtgcatagcgaggtgcagctggtggagagcggcggcggcctggtgcagcccggcaacagcctgaccctgagctgcgtggccagcggcttcaccttcagcaactacggcatgcactggatcaggcaggcccccaagaagggcctggagtggatcgccatgatcgcctacgacagcagcaagatgaactacgccgacaccgtgaagggccgcttcaccatcagccgcgacaacagcaagaacaccctgtacctggagatgaacagcctgcgcagcgaggacaccgccatgtactactgcgccgtgcccaccgcccactacgtggtggacgtgtggggacaaggcgtgagcgtgaccgtgagcagcggtggcggagggtctggcggaggaggttccgggggcggtggaagcgacatccagatgacccagagccccgccagtctgagcgccagcctggaggagatcgtgaccatcacctgccaggcaagccaagacatcggcaactggctggcctggtaccagcagaagcccggcaagagcccccagctgctgatcgccggcgccaccagcctggccgacggcgtgcccagccgcttcagcggcagccgcagcggcacccagttcagcctgaagatcagccgcgtgcaggtggaggacatcggcatctactactgcctgcaggccgccaacaccccctggaccttcggcggcggcaccaagctggagctgaagcgctaataaggtggcggagggtctggaggtggcggatcaggcggaggaggatcttccgaaacgcaggccaactcgaccacagatgctctgaacgttcttctcatcatcgtggatgacctgcgcccctccctgggctgttatggggataagctggtgaggtccccaaatattgaccaactggcatcccacagcctcctcttccagaatgcctttgcgcagcaagcagtgtgcgccccgagccgcgtttctttcctcactggcaggagacctgacaccacccgcctgtacgacttcaactcctactggagggtgcacgctggaaacttctccaccatcccccagtacttcaaggagaatggctatgtgaccatgtcggtgggaaaagtctttcaccctgggatatcttctaaccataccgatgattctccgtatagctggtcttttccaccttatcatccttcctctgagaagtatgaaaacactaagacatgtcgagggccagatggagaactccatgccaacctgctttgccctgtggatgtgctggatgttcccgagggcaccttgcctgacaaacagagcactgagcaagccatacagttgttggaaaagatgaaaacgtcagccagtcctttcttcctggccgttgggtatcataagccacacatccccttcagataccccaaggaatttcagaagttgtatcccttggagaacatcaccctggcccccgatcccgaggtccctgatggcctaccccctgtggcctacaacccctggatggacatcaggcaacgggaagacgtccaagccttaaacatcagtgtgccgtatggtccaattcctgtggactttcagcggaaaatccgccagagctactttgcctctgtgtcatatttggatacacaggtcggccgcctcttgagtgctttggacgatcttcagctggccaacagcaccatcattgcatttacctcggatcatgggtgggctctaggtgaacatggagaatgggccaaatacagcaattttgatgttgctacccatgttcccctgatattctatgttcctggaaggacggcttcacttccggaggcaggcgagaagcttttcccttacctcgacccttttgattccgcctcacagttgatggagccaggcaggcaatccatggaccttgtggaacttgtgtctctttttcccacgctggctggacttgcaggactgcaggttccacctcgctgccccgttccttcatttcacgttgagctgtgcagagaaggcaagaaccttctgaagcattttcgattccgtgacttggaagaagatccgtacctccctggtaatccccgtgaactgattgcctatagccagtatccccggccttcagacatccctcagtggaattctgacaagccgagtttaaaagatataaagatcatgggctattccatacgcaccatagactataggtatactgtgtgggttggcttcaatcctgatgaatttctagctaacttttctgacatccatgcaggggaactgtattttgtggattctgacccattgcaggatcacaatatgtataatgattcccaaggtggagaccttttccagttgttgatgccttaataagcggccgcatttaaatctgtgccttctagttgccagccatctgttgtttgcccctcccccgtgccttccttgaccctggaaggtgccactcccactgtcctttcctaataaaatgaggaaattgcatcgcattgtctgagtaggtgtcattctattctggggggtggggtggggcaggacagcaagggggaggattgggaagacaatagcaggcatgctgggga

SEQ ID NO: 22 - protein, 781 aa, synthetic construct
EVQLVESGGGLVQPGNSLTLSCVASGFTFSNYGMHWIRQAPKKGLEWIAMIAYDSSKMNYADTVKGRFTISRDNSKNTLYLEMNSLRSEDTAMYYCAVPTAHYVVDVWGQGVSVTVSSGGGGSGGGGSGGGGSDIQMTQSPASLSASLEEIVTITCQASQDIGNWLAWYQQKPGKSPQLLIAGATSLADGVPSRFSGSRSGTQFSLKISRVQVEDIGIYYCLQAANTPWTFGGGTKLELKRGGGGSGGGGSGGGGSSETQANSTTDALNVLLIIVDDLRPSLGCYGDKLVRSPNIDQLASHSLLFQNAFAQQAVCAPSRVSFLTGRRPDTTRLYDFNSYWRVHAGNFSTIPQYFKENGYVTMSVGKVFHPGISSNHTDDSPYSWSFPPYHPSSEKYENTKTCRGPDGELHANLLCPVDVLDVPEGTLPDKQSTEQAIQLLEKMKTSASPFFLAVGYHKPHIPFRYPKEFQKLYPLENITLAPDPEVPDGLPPVAYNPWMDIRQREDVQALNISVPYGPIPVDFQRKIRQSYFASVSYLDTQVGRLLSALDDLQLANSTIIAFTSDHGWALGEHGEWAKYSNFDVATHVPLIFYVPGRTASLPEAGEKLFPYLDPFDSASQLMEPGRQSMDLVELVSLFPTLAGLAGLQVPPRCPVPSFHVELCREGKNLLKHFRFRDLEEDPYLPGNPRELIAYSQYPRPSDIPQWNSDKPSLKDIKIMGYSIRTIDYRYTVWVGFNPDEFLANFSDIHAGELYFVDSDPLQDHNMYNDSQGGDLFQLLMP

SEQ ID NO: 23 - DNA, 2403 bp, synthetic construct
  source 1..2403: mol_type = other DNA
atgggctggagctgcattattctgtttctggtggcgaccgcgaccggcgtgcatagcgaggtgcagctggtggagagcggcggcggcctggtgcagcccggcaacagcctgaccctgagctgcgtggccagcggcttcaccttcagcaactacggcatgcactggatcaggcaggcccccaagaagggcctggagtggatcgccatgatcgcctacgacagcagcaagatgaactacgccgacaccgtgaagggccgcttcaccatcagccgcgacaacagcaagaacaccctgtacctggagatgaacagcctgcgcagcgaggacaccgccatgtactactgcgccgtgcccaccgcccactacgtggtggacgtgtggggacaaggcgtgagcgtgaccgtgagcagcggtggcggagggtctggcggaggaggttccgggggcggtggaagcgacatccagatgacccagagccccgccagtctgagcgccagcctggaggagatcgtgaccatcacctgccaggcaagccaagacatcggcaactggctggcctggtaccagcagaagcccggcaagagcccccagctgctgatcgccggcgccaccagcctggccgacggcgtgcccagccgcttcagcggcagccgcagcggcacccagttcagcctgaagatcagccgcgtgcaggtggaggacatcggcatctactactgcctgcaggccgccaacaccccctggaccttcggcggcggcaccaagctggagctgaagcgcggtggcggagggtctggaggtggcggatcaggcggaggaggatcttccgaaacgcaggccaactcgaccacagatgctctgaacgttcttctcatcatcgtggatgacctgcgcccctccctgggctgttatggggataagctggtgaggtccccaaatattgaccaactggcatcccacagcctcctcttccagaatgcctttgcgcagcaagcagtgtgcgccccgagccgcgtttctttcctcactggcaggagacctgacaccacccgcctgtacgacttcaactcctactggagggtgcacgctggaaacttctccaccatcccccagtacttcaaggagaatggctatgtgaccatgtcggtgggaaaagtctttcaccctgggatatcttctaaccataccgatgattctccgtatagctggtcttttccaccttatcatccttcctctgagaagtatgaaaacactaagacatgtcgagggccagatggagaactccatgccaacctgctttgccctgtggatgtgctggatgttcccgagggcaccttgcctgacaaacagagcactgagcaagccatacagttgttggaaaagatgaaaacgtcagccagtcctttcttcctggccgttgggtatcataagccacacatccccttcagataccccaaggaatttcagaagttgtatcccttggagaacatcaccctggcccccgatcccgaggtccctgatggcctaccccctgtggcctacaacccctggatggacatcaggcaacgggaagacgtccaagccttaaacatcagtgtgccgtatggtccaattcctgtggactttcagcggaaaatccgccagagctactttgcctctgtgtcatatttggatacacaggtcggccgcctcttgagtgctttggacgatcttcagctggccaacagcaccatcattgcatttacctcggatcatgggtgggctctaggtgaacatggagaatgggccaaatacagcaattttgatgttgctacccatgttcccctgatattctatgttcctggaaggacggcttcacttccggaggcaggcgagaagcttttcccttacctcgacccttttgattccgcctcacagttgatggagccaggcaggcaatccatggaccttgtggaacttgtgtctctttttcccacgctggctggacttgcaggactgcaggttccacctcgctgccccgttccttcatttcacgttgagctgtgcagagaaggcaagaaccttctgaagcattttcgattccgtgacttggaagaagatccgtacctccctggtaatccccgtgaactgattgcctatagccagtatccccggccttcagacatccctcagtggaattctgacaagccgagtttaaaagatataaagatcatgggctattccatacgcaccatagactataggtatactgtgtgggttggcttcaatcctgatgaatttctagctaacttttctgacatccatgcaggggaactgtattttgtggattctgacccattgcaggatcacaatatgtataatgattcccaaggtggagaccttttccagttgttgatgccttaa

SEQ ID NO: 24 - DNA, 3426 bp, synthetic construct
  source 1..3426: mol_type = other DNA
atcaagcttagatcattttgatggcagagttcagtttaccgggtcacattgtacctgggaagattcaaggatttatggaaaaagtcaacaacaggagtcagagcagccggaaaagcatggactctgtacttaggactgcgctttgagcaatggcacagcaagctataaccctgtttgcagtcagcacacaaactgtggttcaaagctccactttatctcttcttgtggaattcagatatcagatcagttttgctcaaatgggagacaaagagattaagctcttatgtaaaatttgctgttttacataactttaatgaatggacaaagtcttgtgcatgggggtgggggtggggttagaggggaacagctccagatggcaaacatacgcaagggatttagtcaaacaactttttggcaaagatggtatgattttgtaatggggtaggaaccaatgaaatgcgaggtaagtatggttaataatctacagttattggttaaagaagtatattagagcgagtctttctgcacacagatcaccttcctatcaaccccactagcctctggcaaaggtaccagtgtacagggagtcgctgcgttgccttcgccccgtgccccgctccgcgccgcctcgcgccgcccgccccggctctgactgaccgcgttactcccacaggtgagcgggcgggacggcccttctcctccgggctgtaattagcaagaggtaagggtttaagggatggttggttggtggggtattaatgtttaattacctggagcacctgcctgaaatcactttttttcaggttggacgcgtgccgccaccatgccgccaccccggaccggccgaggccttctctggctgggtctggttctgagctccgtctgcgtcgccctcggatccgaaacgcaggccaactcgaccacagatgctctgaacgttcttctcatcatcgtggatgacctgcgcccctccctgggctgttatggggataagctggtgaggtccccaaatattgaccaactggcatcccacagcctcctcttccagaatgcctttgcgcagcaagcagtgtgcgccccgagccgcgtttctttcctcactggcaggagacctgacaccacccgcctgtacgacttcaactcctactggagggtgcacgctggaaacttctccaccatcccccagtacttcaaggagaatggctatgtgaccatgtcggtgggaaaagtctttcaccctgggatatcttctaaccataccgatgattctccgtatagctggtcttttccaccttatcatccttcctctgagaagtatgaaaacactaagacatgtcgagggccagatggagaactccatgccaacctgctttgccctgtggatgtgctggatgttcccgagggcaccttgcctgacaaacagagcactgagcaagccatacagttgttggaaaagatgaaaacgtcagccagtcctttcttcctggccgttgggtatcataagccacacatccccttcagataccccaaggaatttcagaagttgtatcccttggagaacatcaccctggcccccgatcccgaggtccctgatggcctaccccctgtggcctacaacccctggatggacatcaggcaacgggaagacgtccaagccttaaacatcagtgtgccgtatggtccaattcctgtggactttcagcggaaaatccgccagagctactttgcctctgtgtcatatttggatacacaggtcggccgcctcttgagtgctttggacgatcttcagctggccaacagcaccatcattgcatttacctcggatcatgggtgggctctaggtgaacatggagaatgggccaaatacagcaattttgatgttgctacccatgttcccctgatattctatgttcctggaaggacggcttcacttccggaggcaggcgagaagcttttcccttacctcgacccttttgattccgcctcacagttgatggagccaggcaggcaatccatggaccttgtggaacttgtgtctctttttcccacgctggctggacttgcaggactgcaggttccacctcgctgccccgttccttcatttcacgttgagctgtgcagagaaggcaagaaccttctgaagcattttcgattccgtgacttggaagaagatccgtacctccctggtaatccccgtgaactgattgcctatagccagtatccccggccttcagacatccctcagtggaattctgacaagccgagtttaaaagatataaagatcatgggctattccatacgcaccatagactataggtatactgtgtgggttggcttcaatcctgatgaatttctagctaacttttctgacatccatgcaggggaactgtattttgtggattctgacccattgcaggatcacaatatgtataatgattcccaaggtggagaccttttccagttgttgatgcctgaggtgcagctggtggagagcggcggcggcctggtgcagcccggcaacagcctgaccctgagctgcgtggccagcggcttcaccttcagcaactacggcatgcactggatcaggcaggcccccaagaagggcctggagtggatcgccatgatcgcctacgacagcagcaagatgaactacgccgacaccgtgaagggccgcttcaccatcagccgcgacaacagcaagaacaccctgtacctggagatgaacagcctgcgcagcgaggacaccgccatgtactactgcgccgtgcccaccgcccactacgtggtggacgtgtggggacaaggcgtgagcgtgaccgtgagcagcggtggcggagggtctggcggaggaggttccgggggcggtggaagcgacatccagatgacccagagccccgccagtctgagcgccagcctggaggagatcgtgaccatcacctgccaggcaagccaagacatcggcaactggctggcctggtaccagcagaagcccggcaagagcccccagctgctgatcgccggcgccaccagcctggccgacggcgtgcccagccgcttcagcggcagccgcagcggcacccagttcagcctgaagatcagccgcgtgcaggtggaggacatcggcatctactactgcctgcaggccgccaacaccccctggaccttcggcggcggcaccaagctggagctgaagcgctaataagcggccgcatttaaatctgtgccttctagttgccagccatctgttgtttgcccctcccccgtgccttccttgaccctggaaggtgccactcccactgtcctttcctaataaaatgaggaaattgcatcgcattgtctgagtaggtgtcattctattctggggggtggggtggggcaggacagcaagggggaggattgggaagacaatagcaggcatgctgggga

SEQ ID NO: 25 - protein, 766 aa, synthetic construct
SETQANSTTDALNVLLIIVDDLRPSLGCYGDKLVRSPNIDQLASHSLLFQNAFAQQAVCAPSRVSFLTGRRPDTTRLYDFNSYWRVHAGNFSTIPQYFKENGYVTMSVGKVFHPGISSNHTDDSPYSWSFPPYHPSSEKYENTKTCRGPDGELHANLLCPVDVLDVPEGTLPDKQSTEQAIQLLEKMKTSASPFFLAVGYHKPHIPFRYPKEFQKLYPLENITLAPDPEVPDGLPPVAYNPWMDIRQREDVQALNISVPYGPIPVDFQRKIRQSYFASVSYLDTQVGRLLSALDDLQLANSTIIAFTSDHGWALGEHGEWAKYSNFDVATHVPLIFYVPGRTASLPEAGEKLFPYLDPFDSASQLMEPGRQSMDLVELVSLFPTLAGLAGLQVPPRCPVPSFHVELCREGKNLLKHFRFRDLEEDPYLPGNPRELIAYSQYPRPSDIPQWNSDKPSLKDIKIMGYSIRTIDYRYTVWVGFNPDEFLANFSDIHAGELYFVDSDPLQDHNMYNDSQGGDLFQLLMPEVQLVESGGGLVQPGNSLTLSCVASGFTFSNYGMHWIRQAPKKGLEWIAMIAYDSSKMNYADTVKGRFTISRDNSKNTLYLEMNSLRSEDTAMYYCAVPTAHYVVDVWGQGVSVTVSSGGGGSGGGGSGGGGSDIQMTQSPASLSASLEEIVTITCQASQDIGNWLAWYQQKPGKSPQLLIAGATSLADGVPSRFSGSRSGTQFSLKISRVQVEDIGIYYCLQAANTPWTFGGGTKLELKR

SEQ ID NO: 26 - DNA, 2376 bp, synthetic construct
  source 1..2376: mol_type = other DNA
atgccgccaccccggaccggccgaggccttctctggctgggtctggttctgagctccgtctgcgtcgccctcggatccgaaacgcaggccaactcgaccacagatgctctgaacgttcttctcatcatcgtggatgacctgcgcccctccctgggctgttatggggataagctggtgaggtccccaaatattgaccaactggcatcccacagcctcctcttccagaatgcctttgcgcagcaagcagtgtgcgccccgagccgcgtttctttcctcactggcaggagacctgacaccacccgcctgtacgacttcaactcctactggagggtgcacgctggaaacttctccaccatcccccagtacttcaaggagaatggctatgtgaccatgtcggtgggaaaagtctttcaccctgggatatcttctaaccataccgatgattctccgtatagctggtcttttccaccttatcatccttcctctgagaagtatgaaaacactaagacatgtcgagggccagatggagaactccatgccaacctgctttgccctgtggatgtgctggatgttcccgagggcaccttgcctgacaaacagagcactgagcaagccatacagttgttggaaaagatgaaaacgtcagccagtcctttcttcctggccgttgggtatcataagccacacatccccttcagataccccaaggaatttcagaagttgtatcccttggagaacatcaccctggcccccgatcccgaggtccctgatggcctaccccctgtggcctacaacccctggatggacatcaggcaacgggaagacgtccaagccttaaacatcagtgtgccgtatggtccaattcctgtggactttcagcggaaaatccgccagagctactttgcctctgtgtcatatttggatacacaggtcggccgcctcttgagtgctttggacgatcttcagctggccaacagcaccatcattgcatttacctcggatcatgggtgggctctaggtgaacatggagaatgggccaaatacagcaattttgatgttgctacccatgttcccctgatattctatgttcctggaaggacggcttcacttccggaggcaggcgagaagcttttcccttacctcgacccttttgattccgcctcacagttgatggagccaggcaggcaatccatggaccttgtggaacttgtgtctctttttcccacgctggctggacttgcaggactgcaggttccacctcgctgccccgttccttcatttcacgttgagctgtgcagagaaggcaagaaccttctgaagcattttcgattccgtgacttggaagaagatccgtacctccctggtaatccccgtgaactgattgcctatagccagtatccccggccttcagacatccctcagtggaattctgacaagccgagtttaaaagatataaagatcatgggctattccatacgcaccatagactataggtatactgtgtgggttggcttcaatcctgatgaatttctagctaacttttctgacatccatgcaggggaactgtattttgtggattctgacccattgcaggatcacaatatgtataatgattcccaaggtggagaccttttccagttgttgatgcctgaggtgcagctggtggagagcggcggcggcctggtgcagcccggcaacagcctgaccctgagctgcgtggccagcggcttcaccttcagcaactacggcatgcactggatcaggcaggcccccaagaagggcctggagtggatcgccatgatcgcctacgacagcagcaagatgaactacgccgacaccgtgaagggccgcttcaccatcagccgcgacaacagcaagaacaccctgtacctggagatgaacagcctgcgcagcgaggacaccgccatgtactactgcgccgtgcccaccgcccactacgtggtggacgtgtggggacaaggcgtgagcgtgaccgtgagcagcggtggcggagggtctggcggaggaggttccgggggcggtggaagcgacatccagatgacccagagccccgccagtctgagcgccagcctggaggagatcgtgaccatcacctgccaggcaagccaagacatcggcaactggctggcctggtaccagcagaagcccggcaagagcccccagctgctgatcgccggcgccaccagcctggccgacggcgtgcccagccgcttcagcggcagccgcagcggcacccagttcagcctgaagatcagccgcgtgcaggtggaggacatcggcatctactactgcctgcaggccgccaacaccccctggaccttcggcggcggcaccaagctggagctgaagcgctaa

SEQ ID NO: 27 - DNA, 2727 bp, synthetic construct
  source 1..2727: mol_type = other DNA
atcgatatcaagcttagatcattttgatggcagagttcagtttaccgggtcacattgtacctgggaagattcaaggatttatggaaaaagtcaacaacaggagtcagagcagccggaaaagcatggactctgtacttaggactgcgctttgagcaatggcacagcaagctataaccctgtttgcagtcagcacacaaactgtggttcaaagctccactttatctcttcttgtggaattcagatatcagatcagttttgctcaaatgggagacaaagagattaagctcttatgtaaaatttgctgttttacataactttaatgaatggacaaagtcttgtgcatgggggtgggggtggggttagaggggaacagctccagatggcaaacatacgcaagggatttagtcaaacaactttttggcaaagatggtatgattttgtaatggggtaggaaccaatgaaatgcgaggtaagtatggttaataatctacagttattggttaaagaagtatattagagcgagtctttctgcacacagatcaccttcctatcaaccccactagcctctggcaaaggtaccagtgtacagggagtcgctgcgttgccttcgccccgtgccccgctccgcgccgcctcgcgccgcccgccccggctctgactgaccgcgttactcccacaggtgagcgggcgggacggcccttctcctccgggctgtaattagcaagaggtaagggtttaagggatggttggttggtggggtattaatgtttaattacctggagcacctgcctgaaatcactttttttcaggttggacgcgtggtacctctagagtcgaggccaccatgccgccaccccggaccggccgaggccttctctggctgggtctggttctgagctccgtctgcgtcgccctcggatccgaaacgcaggccaactcgaccacagatgctctgaacgttcttctcatcatcgtggatgacctgcgcccctccctgggctgttatggggataagctggtgaggtccccaaatattgaccaactggcatcccacagcctcctcttccagaatgcctttgcgcagcaagcagtgtgcgccccgagccgcgtttctttcctcactggcaggagacctgacaccacccgcctgtacgacttcaactcctactggagggtgcacgctggaaacttctccaccatcccccagtacttcaaggagaatggctatgtgaccatgtcggtgggaaaagtctttcaccctgggatatcttctaaccataccgatgattctccgtatagctggtcttttccaccttatcatccttcctctgagaagtatgaaaacactaagacatgtcgagggccagatggagaactccatgccaacctgctttgccctgtggatgtgctggatgttcccgagggcaccttgcctgacaaacagagcactgagcaagccatacagttgttggaaaagatgaaaacgtcagccagtcctttcttcctggccgttgggtatcataagccacacatccccttcagataccccaaggaatttcagaagttgtatcccttggagaacatcaccctggcccccgatcccgaggtccctgatggcctaccccctgtggcctacaacccctggatggacatcaggcaacgggaagacgtccaagccttaaacatcagtgtgccgtatggtccaattcctgtggactttcagcggaaaatccgccagagctactttgcctctgtgtcatatttggatacacaggtcggccgcctcttgagtgctttggacgatcttcagctggccaacagcaccatcattgcatttacctcggatcatgggtgggctctaggtgaacatggagaatgggccaaatacagcaattttgatgttgctacccatgttcccctgatattctatgttcctggaaggacggcttcacttccggaggcaggcgagaagcttttcccttacctcgacccttttgattccgcctcacagttgatggagccaggcaggcaatccatggaccttgtggaacttgtgtctctttttcccacgctggctggacttgcaggactgcaggttccacctcgctgccccgttccttcatttcacgttgagctgtgcagagaaggcaagaaccttctgaagcattttcgattccgtgacttggaagaagatccgtacctccctggtaatccccgtgaactgattgcctatagccagtatccccggccttcagacatccctcagtggaattctgacaagccgagtttaaaagatataaagatcatgggctattccatacgcaccatagactataggtatactgtgtgggttggcttcaatcctgatgaatttctagctaacttttctgacatccatgcaggggaactgtattttgtggattctgacccattgcaggatcacaatatgtataatgattcccaaggtggggatcttttccagttgttgatgccttgagcggccgcatttaaatctgtgccttctagttgccagccatctgttgtttgcccctcccccgtgccttccttgaccctggaaggtgccactcccactgtcctttcctaataaaatgaggaaattgcatcgcattgtctgagtaggtgtcattctattctggggggtggggtggggcaggacagcaagggggaggattgggaagacaatagcaggcatgctggggaagatct

SEQ ID NO: 28 - DNA, 1589 bp, Homo sapiens
  source 1..1589: mol_type = genomic DNA
tccgaaacgcaggccaactcgaccacagatgctctgaacgttcttctcatcatcgtggatgacctgcgcccctccctgggctgttatggggataagctggtgaggtccccaaatattgaccaactggcatcccacagcctcctcttccagaatgcctttgcgcagcaagcagtgtgcgccccgagccgcgtttctttcctcactggcaggagacctgacaccacccgcctgtacgacttcaactcctactggagggtgcacgctggaaacttctccaccatcccccagtacttcaaggagaatggctatgtgaccatgtcggtgggaaaagtctttcaccctgggatatcttctaaccataccgatgattctccgtatagctggtcttttccaccttatcatccttcctctgagaagtatgaaaacactaagacatgtcgagggccagatggagaactccatgccaacctgctttgccctgtggatgtgctggatgttcccgagggcaccttgcctgacaaacagagcactgagcaagccatacagttgttggaaaagatgaaaacgtcagccagtcctttcttcctggccgttgggtatcataagccacacatccccttcagataccccaaggaatttcagaagttgtatcccttggagaacatcaccctggcccccgatcccgaggtccctgatggcctaccccctgtggcctacaacccctggatggacatcaggcaacgggaagacgtccaagccttaaacatcagtgtgccgtatggtccaattcctgtggactttcagcggaaaatccgccagagctactttgcctctgtgtcatatttggatacacaggtcggccgcctcttgagtgctttggacgatcttcagctggccaacagcaccatcattgcatttacctcggatcatgggtgggctctaggtgaacatggagaatgggccaaatacagcaattttgatgttgctacccatgttcccctgatattctatgttcctggaaggacggcttcacttccggaggcaggcgagaagcttttcccttacctcgacccttttgattccgcctcacagttgatggagccaggcaggcaatccatggaccttgtggaacttgtgtctctttttcccacgctggctggacttgcaggactgcaggttccacctcgctgccccgttccttcatttcacgttgagctgtgcagagaaggcaagaaccttctgaagcattttcgattccgtgacttggaagaagatccgtacctccctggtaatccccgtgaactgattgcctatagccagtatccccggccttcagacatccctcagtggaattctgacaagccgagtttaaaagatataaagatcatgggctattccatacgcaccatagactataggtatactgtgtgggttggcttcaatcctgatgaatttctagctaacttttctgacatccatgcaggggaactgtattttgtggattctgacccattgcaggatcacaatatgtataatgattcccaaggtggagaccttttccagttgttgatgccttaataagcggccgc

SEQ ID NO: 29 - DNA, 2820 bp, synthetic construct
  source 1..2820: mol_type = other DNA
agcgctcggaccgggcgcgctcactggccgtcgttttacaacgtcgtgactgggaaaaccctgtacaggctgaccggtgttgcctaggtgaatggcgaatggtcaggtggcacttttcggggaaatgtgcgcggaacccctatttgtttatttttctaaatacattcaaatatgtatccgctcatgagacaataaccctgataaatgcttcaataatattgaaaaaggaagagtatgagtattcaacatttccgtgtcgcccttattcccttttttgcggcattttgccttcctgtttttgctcacccagaaacgctggtgaaagtaaaagatgctgaagatcagttgggtgcacgagtgggttacatcgaactggatctcaacagcggtaagatccttgagagttttcgccccgaagaacgttttccaatgatgagcacttttaaagttctgctatgtggcgcggtattatcccgtattgacgccgggcaagagcaactcggtcgccgcatacactattctcagaatgacttggttgagtactcaccagtcacagaaaagcatcttacggatggcatgacagtaagagaattatgcagtgctgccataaccatgagtgataacactgcggccaacttacttctgacaacgatcggaggaccgaaggagctaaccgcttttttgcacaacatgggggatcatgtaactcgccttgatcgttgggaaccggagctgaatgaagccataccaaacgacgagcgtgacaccacgatgcctgtagcaatggcaacaacgttgcgcaaactattaactggcgaactacttactctagcttcccggcaacaattaatagactggatggaggcggataaagttgcaggaccacttctgcgctcggcccttccggctggctggtttattgctgataaatctggagccggtgagcgtgggtctcgcggtatcattgcagcactggggccagatggtaagccctcccgtatcgtagttatctacacgacggggagtcaggcaactatggatgaacgaaatagacagatcgctgagataggtgcctcactgattaagcattggtaactgtcagaccaagtttactcatatatactttagattgatttaaaacttcatttttaatttaaaaggatctaggtgaagatcctttttgataatctcatgaccaaaatcccttaacgtgagttttcgttccactgagcgtcagaccccgtagaaaagatcaaaggatcttcttgagatcctttttttctgcgcgtaatctgctgcttgcaaacaaaaaaaccaccgctaccagcggtggtttgtttgccggatcaagagctaccaactctttttccgaaggtaactggcttcagcagagcgcagataccaaatactgttcttctagtgtagccgtagttaggccaccacttcaagaactctgtagcaccgcctacatacctcgctctgctaatcctgttaccagtggctgctgccagtggcgataagtcgtgtcttaccgggttggactcaagacgatagttaccggataaggcgcagcggtcgggctgaacggggggttcgtgcacacagcccagcttggagcgaacgacctacaccgaactgagatacctacagcgtgagctatgagaaagcgccacgcttcccgaagggagaaaggcggacaggtatccggtaagcggcagggtcggaacaggagagcgcacgagggagcttccagggggaaacgcctggtatctttatagtcctgtcgggtttcgccacctctgacttgagcgtcgatttttgtgatgctcgtcaggggggcggagcctatggaaaaacgccagcaacgcggcctttttacggttcctggccttttgctggccttttgctcacatgttctttcctgcgttatcccctgattctgtggataaccgtattaccgcctttgagtgagctgataccgctcgccgcagccgaacgaccgagcgcagcgagtcagtgagcgaggaagcggaagagcgcccaatacgcaaaccgcctctccccgcgcgttggccgattcattaatgcagctggcacgacaggtttcccgactggaaagcgggcagtgagcgcaacgcaattaatgtgagttagctcactcattaggcaccccaggctttacactttatgcttccggctcgtatgttgtgtggaattgtgagcggataacaatttcacacaggaaacagctatgaccatgattacgccaacggaccgggaggggtggagtcgtgacgtgaattacgtcatagggttagggaggtcctgtattagaggtcacgtgagtgttttgcgacattttgcgacaccatgtggtctcgctgggggggggggcccgagtgagcacgcagggtctccattttgaagcgggaggtttgaacgcgcagccgccacgccggggttttacgagattgtgattaaggtccccagcgaccttgacgagcatctgcccggcatttctgacagctttgtgaactgggtggccgagaaggaatgggagttgccgccagattctgacatggatctgaatctgattgagcaggcacccctgaccgtggccgagaagctgcagcgcgactttctgacggaatggcgccgtgtgagtaaggccccggaggcccttttctttgtgcaatttgagaagggagagagctacttccacatgcacgtgctcgtggaaaccaccggggtgaaatccatggttttgggacgtttcctgagtcagattcgcgaaaaactgattcagagaatttaccgcgg

SEQ ID NO: 30 - DNA, 2911 bp, synthetic construct
  source 1..2911: mol_type = other DNA
aagcttcgatcaactacgcagacaggtaccaaaacaaatgttctcgtcacgtgggcatgaatctgatgctgtttccctgcagacaatgcgagagaatgaatcagaattcaaatatctgcttcactcacggacagaaagactgtttagagtgctttcccgtgtcagaatctcaacccgtttctgtcgtcaaaaaggcgtatcagaaactgtgctacattcatcatatcatgggaaaggtgccagacgcttgcactgcctgcgatctggtcaatgtggatttggatgactgcatctttgaacaataaatgatttaaatcaggtatggctgccgatggttatcttccagattggctcgaggacaacctctctgagggcattcgcgagtggtgggacttgaaacctggagccccgaaacccaaagccaaccagcaaaagcaggacgacggccggggtctggtgcttcctggctacaagtacctcggacccttcaacggactcgacaagggggagcccgtcaacgcggcggatgcagcggccctcgagcacgacaaggcctacgaccagcagctcaaagcgggtgacaatccgtacctgcggtataaccacgccgacgccgagtttcaggagcgtctgcaagaagatacgtcttttgggggcaacctcgggcgagcagtcttccaggccaagaagagggttctcgaaccttttggtctggttgaggaaggtgctaagacggctcctggaaagaaacgtccggtagagcagtcgccacaagagccagactcctcctcgggcattggcaagacaggccagcagcccgctaaaaagagactcaattttggtcagactggcgactcagagtcagtccccgacccacaacctctcggagaacctccagcaacccccgctgctgtgggacctactacaatggcttcaggcggtggcgcaccaatggcagacaataacgaaggcgccgacggagtgggtaatgcctcaggaaattggcattgcgattccacatggctgggcgacagagtcatcaccaccagcacccgaacatgggccttgcccacctataacaaccacctctacaagcaaatctccagtgcttcaacgggggccagcaacgacaaccactacttcggctacagcaccccctgggggtattttgatttcaacagattccactgccatttctcaccacgtgactggcagcgactcatcaacaacaattggggattccggcccaagagactcaacttcaagctcttcaacatccaagtcaaggaggtcacgacgaatgatggcgtcacgaccatcgctaataaccttaccagcacggttcaagtcttctcggactcggagtaccagttgccgtacgtcctcggctctgcgcaccagggctgcctccctccgttcccggcggacgtgttcatgattccgcagtacggctacctaacgctcaacaatggcagccaggcagtgggacggtcatccttttactgcctggaatatttcccatcgcagatgctgagaacgggcaataactttaccttcagctacaccttcgaggacgtgcctttccacagcagctacgcgcacagccagagcctggaccggctgatgaatcctctcatcgaccagtacctgtattacctgaacagaactcagaatcagtccggaagtgcccaaaacaaggacttgctgtttagccgggggtctccagctggcatgtctgttcagcccaaaaactggctacctggaccctgttaccggcagcagcgcgtttctaaaacaaaaacagacaacaacaacagcaactttacctggactggtgcttcaaaatataaccttaatgggcgtgaatctataatcaaccctggcactgctatggcctcacacaaagacgacaaagacaagttctttcccatgagcggtgtcatgatttttggaaaggagagcgccggagcttcaaacactgcattggacaatgtcatgatcacagacgaagaggaaatcaaagccactaaccccgtggccaccgaaagatttgggactgtggcagtcaatctccagagcagcagcacagaccctgcgaccggagatgtgcatgttatgggagccttacctggaatggtgtggcaagacagagacgtatacctgcagggtcctatttgggccaaaattcctcacacggatggacactttcacccgtctcctctcatgggcggctttggacttaagcacccgcctcctcagatcctcatcaaaaacacgcctgttcctgcgaatcctccggcagagttttcggctacaaagtttgcttcattcatcacccagtattccacaggacaagtgagcgtggagattgaatgggagctgcagaaagaaaacagcaaacgctggaatcccgaagtgcagtatacatctaactatgcaaaatctgccaacgttgatttcactgtggacaacaatggactttatactgagcctcgccccattggcacccgttacctcacccgtcccctgtaattgcttgttaatcaataaaccgtttaattcgtttcagttgaactttggtctctgcgtatttctttcttatctagtttccatggctacgtagataagtagcatggcgggttaatcattaactacagcccgggcgtttaaacagcgggcggaggggtggagtcgtgacgtgaattacgtcatagggttagggaggtcctgtattagaggtcacgtgagtgttttgcgacattttgcgacaccatgtggtctcgctgggggggggggcccgagtgagcacgcagggtctccattttgaagcgggaggtttgaacgagcgctcggaccgggcgcgctcactggccgtcgttttacaacgtcgtgactgggaaaaccctgtaca

SEQ ID NO: 31 - DNA, 2214 bp, Adeno-associated virus serotype 8
  source 1..2214: mol_type = genomic DNA
atggctgccgatggttatcttccagattggctcgaggacaacctctctgagggcattcgcgagtggtgggcgctgaaacctggagccccgaagcccaaagccaaccagcaaaagcaggacgacggccggggtctggtgcttcctggctacaagtacctcggacccttcaacggactcgacaagggggagcccgtcaacgcggcggacgcagcggccctcgagcacgacaaggcctacgaccagcagctgcaggcgggtgacaatccgtacctgcggtataaccacgccgacgccgagtttcaggagcgtctgcaagaagatacgtcttttgggggcaacctcgggcgagcagtcttccaggccaagaagcgggttctcgaacctctcggtctggttgaggaaggcgctaagacggctcctggaaagaagagaccggtagagccatcaccccagcgttctccagactcctctacgggcatcggcaagaaaggccaacagcccgccagaaaaagactcaattttggtcagactggcgactcagagtcagttccagaccctcaacctctcggagaacctccagcagcgccctctggtgtgggacctaatacaatggctgcaggcggtggcgcaccaatggcagacaataacgaaggcgccgacggagtgggtagttcctcgggaaattggcattgcgattccacatggctgggcgacagagtcatcaccaccagcacccgaacctgggccctgcccacctacaacaaccacctctacaagcaaatctccaacgggacatcgggaggagccaccaacgacaacacctacttcggctacagcaccccctgggggtattttgactttaacagattccactgccacttttcaccacgtgactggcagcgactcatcaacaacaactggggattccggcccaagagactcagcttcaagctcttcaacatccaggtcaaggaggtcacgcagaatgaaggcaccaagaccatcgccaataacctcaccagcaccatccaggtgtttacggactcggagtaccagctgccgtacgttctcggctctgcccaccagggctgcctgcctccgttcccggcggacgtgttcatgattccccagtacggctacctaacactcaacaacggtagtcaggccgtgggacgctcctccttctactgcctggaatactttccttcgcagatgctgagaaccggcaacaacttccagtttacttacaccttcgaggacgtgcctttccacagcagctacgcccacagccagagcttggaccggctgatgaatcctctgattgaccagtacctgtactacttgtctcggactcaaacaacaggaggcacggcaaatacgcagactctgggcttcagccaaggtgggcctaatacaatggccaatcaggcaaagaactggctgccaggaccctgttaccgccaacaacgcgtctcaacgacaaccgggcaaaacaacaatagcaactttgcctggactgctgggaccaaataccatctgaatggaagaaattcattggctaatcctggcatcgctatggcaacacacaaagacgacgaggagcgtttttttcccagtaacgggatcctgatttttggcaaacaaaatgctgccagagacaatgcggattacagcgatgtcatgctcaccagcgaggaagaaatcaaaaccactaaccctgtggctacagaggaatacggtatcgtggcagataacttgcagcagcaaaacacggctcctcaaattggaactgtcaacagccagggggccttacccggtatggtctggcagaaccgggacgtgtacctgcagggtcccatctgggccaagattcctcacacggacggcaacttccacccgtctccgctgatgggcggctttggcctgaaacatcctccgcctcagatcctgatcaagaacacgcctgtacctgcggatcctccgaccaccttcaaccagtcaaagctgaactctttcatcacgcaatacagcaccggacaggtcagcgtggaaattgaatgggagctgcagaaggaaaacagcaagcgctggaaccccgagatccagtacacctccaactactacaaatctacaagtgtggactttgctgttaatacagaaggcgtgtactctgaaccccgccccattggcacccgttacctcacccgtaatctg

SEQ ID NO: 32 - DNA, 1866 bp, Adeno-associated virus serotype 2
  source 1..1866: mol_type = genomic DNA
acgccggggttttacgagattgtgattaaggtccccagcgaccttgacgagcatctgcccggcatttctgacagctttgtgaactgggtggccgagaaggaatgggagttgccgccagattctgacatggatctgaatctgattgagcaggcacccctgaccgtggccgagaagctgcagcgcgactttctgacggaatggcgccgtgtgagtaaggccccggaggcccttttctttgtgcaatttgagaagggagagagctacttccacatgcacgtgctcgtggaaaccaccggggtgaaatccatggttttgggacgtttcctgagtcagattcgcgaaaaactgattcagagaatttaccgcgggatcgagccgactttgccaaactggttcgcggtcacaaagaccagaaatggcgccggaggcgggaacaaggtggtggatgagtgctacatccccaattacttgctccccaaaacccagcctgagctccagtgggcgtggactaatatggaacagtatttaagcgcctgtttgaatctcacggagcgtaaacggttggtggcgcagcatctgacgcacgtgtcgcagacgcaggagcagaacaaagagaatcagaatcccaattctgatgcgccggtgatcagatcaaaaacttcagccaggtacatggagctggtcgggtggctcgtggacaaggggattacctcggagaagcagtggatccaggaggaccaggcctcatacatctccttcaatgcggcctccaactcgcggtcccaaatcaaggctgccttggacaatgcgggaaagattatgagcctgactaaaaccgcccccgactacctggtgggccagcagcccgtggaggacatttccagcaatcggatttataaaattttggaactaaacgggtacgatccccaatatgcggcttccgtctttctgggatgggccacgaaaaagttcggcaagaggaacaccatctggctgtttgggcctgcaactaccgggaagaccaacatcgcggaggccatagcccacactgtgcccttctacgggtgcgtaaactggaccaatgagaactttcccttcaacgactgtgtcgacaagatggtgatctggtgggaggaggggaagatgaccgccaaggtcgtggagtcggccaaagccattctcggaggaagcaaggtgcgcgtggaccagaaatgcaagtcctcggcccagatagacccgactcccgtgatcgtcacctccaacaccaacatgtgcgccgtgattgacgggaactcaacgaccttcgaacaccagcagccgttgcaagaccggatgttcaaatttgaactcacccgccgtctggatcatgactttgggaaggtcaccaagcaggaagtcaaagactttttccggtgggcaaaggatcacgtggttgaggtggagcatgaattctacgtcaaaaagggtggagccaagaaaagacccgcccccagtgacgcagatataagtgagcccaaacgggtgcgcgagtcagttgcgcagccatcgacgtcagacgcggaagcttcgatcaactacgcagacaggtaccaaaacaaatgttctcgtcacgtgggcatgaatctgatgctgtttccctgcagacaatgcgagagaatgaatcagaattcaaatatctgcttcactcacggacagaaagactgtttagagtgctttcccgtgtcagaatctcaacccgtttctgtcgtcaaaaaggcgtatcagaaactgtgctacattcatcatatcatgggaaaggtgccagacgcttgcactgcctgcgatctggtcaatgtggatttggatgactgcatctttgaacaataa

SEQ ID NO: 33 - DNA, 16 bp, synthetic construct
  source 1..16: mol_type = other DNA
gccagccatctgttgt

SEQ ID NO: 34 - DNA, 16 bp, synthetic construct
  source 1..16: mol_type = other DNA
ggagtggcaccttcca

SEQ ID NO: 35 - DNA, 21 bp, synthetic construct
  source 1..21: mol_type = other DNA
tcccccgtgccttccttgacc

SEQ ID NO: 36 - DNA, 21 bp, synthetic construct
  source 1..21: mol_type = other DNA
ggaacccctagtgatggagtt

SEQ ID NO: 37 - DNA, 16 bp, synthetic construct
  source 1..16: mol_type = other DNA
cggcctcagtgagcga

SEQ ID NO: 38 - DNA, 21 bp, synthetic construct
  source 1..21: mol_type = other DNA
cactccctctctgcgcgctcg

SEQ ID NO: 39 - protein, 763 aa, Mus musculus
MMDQARSAFSNLFGGEPLSYTRFSLARQVDGDNSHVEMKLAADEEENADNNMKASVRKPKRFNGRLCFAAIALVIFFLIGFMSGYLGYCKRVEQKEECVKLAETEETDKSETMETEDVPTSSRLYWADLKTLLSEKLNSIEFADTIKQLSQNTYTPREAGSQKDESLAYYIENQFHEFKFSKVWRDEHYVKIQVKSSIGQNMVTIVQSNGNLDPVESPEGYVAFSKPTEVSGKLVHANFGTKKDFEELSYSVNGSLVIVRAGEITFAEKVANAQSFNAIGVLIYMDKNKFPVVEADLALFGHAHLGTGDPYTPGFPSFNHTQFPPSQSSGLPNIPVQTISRAAAEKLFGKMEGSCPARWNIDSSCKLELSQNQNVKLIVKNVLKERRILNIFGVIKGYEEPDRYVVVGAQRDALGAGVAAKSSVGTGLLLKLAQVFSDMISKDGFRPSRSIIFASWTAGDFGAVGATEWLEGYLSSLHLKAFTYINLDKVVLGTSNFKVSASPLLYTLMGKIMQDVKHPVDGKSLYRDSNWISKVEKLSFDNAAYPFLAYSGIPAVSFCFCEDADYPYLGTRLDTYEALTQKVPQLNQMVRTAAEVAGQLIIKLTHDVELNLDYEMYNSKLLSFMKDLNQFKTDIRDMGLSLQWLYSARGDYFRATSRLTTDFHNAEKTNRFVMREINDRIMKVEYHFLSPYVSPRESPFRHIFWGSGSHTLSALVENLKLRQKNITAFNETLFRNQLALATWTIQGVANALSGDIWNIDNEF

SEQ ID NO: 40 - protein, 11 aa, synthetic construct
QSLVHSNGNTY

SEQ ID NO: 41 - protein, 16 aa, synthetic construct
RSSQSLVHSNGNTYLH

SEQ ID NO: 42 - protein, 6 aa, synthetic construct
KVSNRF

SEQ ID NO: 43 - protein, 7 aa, synthetic construct
KVSNRFS

SEQ ID NO: 44 - protein, 9 aa, synthetic construct
SQSTHVPWT

SEQ ID NO: 45 - protein, 5 aa, synthetic construct
NYWLG

SEQ ID NO: 46 - protein, 8 aa, synthetic construct
GYSFMNYW

SEQ ID NO: 47 - protein, 8 aa, synthetic construct
IYPGGDYP

SEQ ID NO: 48 - protein, 17 aa, synthetic construct
DIYPGGDYPTYSEKFKV

SEQ ID NO: 49 - protein, 9 aa, synthetic construct
SGNYDEVAY

SEQ ID NO: 50 - protein, 11 aa, synthetic construct
ARSGNYDEVAY

SEQ ID NO: 51 - protein, 766 aa, synthetic construct
EVQLVQSGAEVKKPGESLKISCKGSGYSFMNYWLGWVRQMPGKGLEWMGDIYPGGDYPTYSEKFKVQVTISADKSISTAYLQLSSLKASDTAMYYCARSGNYDEVAYWGQGTLVTVSSASTKGPSVFPLAPSSKSTSGGTAALGCLVKDYFPEPVTVSWNSGALTSGVHTFPAVLQSSGLYSLSSVVTVPSSSLGTQTYICNVNHKPSNTKVDKKVEPKSCDKTHTGGGGSGGGGSGGGGSSETQANSTTDALNVLLIIVDDLRPSLGCYGDKLVRSPNIDQLASHSLLFQNAFAQQAVCAPSRVSFLTGRRPDTTRLYDFNSYWRVHAGNFSTIPQYFKENGYVTMSVGKVFHPGISSNHTDDSPYSWSFPPYHPSSEKYENTKTCRGPDGELHANLLCPVDVLDVPEGTLPDKQSTEQAIQLLEKMKTSASPFFLAVGYHKPHIPFRYPKEFQKLYPLENITLAPDPEVPDGLPPVAYNPWMDIRQREDVQALNISVPYGPIPVDFQRKIRQSYFASVSYLDTQVGRLLSALDDLQLANSTIIAFTSDHGWALGEHGEWAKYSNFDVATHVPLIFYVPGRTASLPEAGEKLFPYLDPFDSASQLMEPGRQSMDLVELVSLFPTLAGLAGLQVPPRCPVPSFHVELCREGKNLLKHFRFRDLEEDPYLPGNPRELIAYSQYPRPSDIPQWNSDKPSLKDIKIMGYSIRTIDYRYTVWVGFNPDEFLANFSDIHAGELYFVDSDPLQDHNMYNDSQGGDLFQLLMP

SEQ ID NO: 52 - DNA, 589 bp, synthetic construct
  source 1..589: mol_type = other DNA
tttgaaagaccccacccgtaggtggcaagctagcttaagtaacgccactttgcaaggcatggaaaaatacataactgagaatagaaaagttcagatcaaggtcaggaacaaagaaacagctgaataccaaacaggatatctgtggtaagcggttcctgccccggctcagggccaagaacagatgagacagctgagtgatgggccaaacaggatatctgtggtaagcagttcctgccccggctcggggccaagaacagatggtccccagatgcggtccagccctcagcagtttctagtgaatcatcagatgtttccagggtgccccaaggacctgaaaatgaccctgtaccttatttgaactaaccaatcagttcgcttctcgcttctgttcgcgcgcttccgctctccgagctcaataaaagagcccacaacccctcactcggcgcgccagtcttccgatagactgcgtcgcccgggtacccgtattcccaataaagcctcttgctgtttgcatccgaatcgtggtctcgctgttccttgggagggtctcctctgagtgattgactacccacgacgggggtctttcatt

SEQ ID NO: 53 - DNA, 594 bp, synthetic construct
  source 1..594: mol_type = other DNA
aatgaaagaccccacctgtaggtttggcaagctagcttaagtaacgccattttgcaaggcatggaaaaatacataactgagaatagagaagttcagatcaaggtcaggaacagatggaacagctgaatatgggccaaacaggatatctgtggtaagcagttcctgccccggctcagggccaagaacagatggaacagctgaatatgggccaaacaggatatctgtggtaagcagttcctgccccggctcagggccaagaacagatggtccccagatgcggtccagccctcagcagtttctagagaaccatcagatgtttccagggtgccccaaggacctgaaatgaccctgtgccttatttgaactaaccaatcagttcgcttctcgcttctgttcgcgcgcttctgctccccgagctcaataaaagagcccacaacccctcactcggggcgccagtcctccgattgactgagtcgcccgggtacccgtgtatccaataaaccctcttgcagttgcatccgacttgtggtctcgctgttccttgggagggtctcctctgagtgattgactacccgtcagcgggggtctttcatt

SEQ ID NO: 54 - DNA, 52 bp, Sendai virus
  source 1..52: mol_type = genomic DNA
accaaacaagagaagaaacttgtttggaatatataatgaagttagacaggat

SEQ ID NO: 55 - DNA, 54 bp, Sendai virus
  source 1..54: mol_type = genomic DNA
acaaggagacaagaaaatttgaaagaataaatatctcttaaactcttgtctggt

SEQ ID NO: 56 - protein, 781 aa, synthetic construct
EVQLVESGGGLVQPGNSLTLSCVASGFTFSNYGMHWIRQAPKKGLEWIAMIAYDSSKMNYADTVKGRFTISRDNSKNTLYLEMNSLRSEDTAMYYCAVPTAHYVVDVWGQGVSVTVSSGGGGSGGGGSGGGGSDIQMTQSPASLSASLEEIVTITCQASQDIGNWLAWYQQKPGKSPQLLIYGATSLADGVPSRFSGSRSGTQFSLKISRVQVEDIGIYYCLQAYNTPWTFGGGTKLELKRGGGGSGGGGSGGGGSSETQANSTTDALNVLLIIVDDLRPSLGCYGDKLVRSPNIDQLASHSLLFQNAFAQQAVCAPSRVSFLTGRRPDTTRLYDFNSYWRVHAGNFSTIPQYFKENGYVTMSVGKVFHPGISSNHTDDSPYSWSFPPYHPSSEKYENTKTCRGPDGELHANLLCPVDVLDVPEGTLPDKQSTEQAIQLLEKMKTSASPFFLAVGYHKPHIPFRYPKEFQKLYPLENITLAPDPEVPDGLPPVAYNPWMDIRQREDVQALNISVPYGPIPVDFQRKIRQSYFASVSYLDTQVGRLLSALDDLQLANSTIIAFTSDHGWALGEHGEWAKYSNFDVATHVPLIFYVPGRTASLPEAGEKLFPYLDPFDSASQLMEPGRQSMDLVELVSLFPTLAGLAGLQVPPRCPVPSFHVELCREGKNLLKHFRFRDLEEDPYLPGNPRELIAYSQYPRPSDIPQWNSDKPSLKDIKIMGYSIRTIDYRYTVWVGFNPDEFLANFSDIHAGELYFVDSDPLQDHNMYNDSQGGDLFQLLMP

SEQ ID NO: 57 - DNA, 3465 bp, synthetic construct
  source 1..3465: mol_type = other DNA
atcgatatcaagcttagatcattttgatggcagagttcagtttaccgggtcacattgtacctgggaagattcaaggatttatggaaaaagtcaacaacaggagtcagagcagccggaaaagcatggactctgtacttaggactgcgctttgagcaatggcacagcaagctataaccctgtttgcagtcagcacacaaactgtggttcaaagctccactttatctcttcttgtggaattcagatatcagatcagttttgctcaaatgggagacaaagagattaagctcttatgtaaaatttgctgttttacataactttaatgaatggacaaagtcttgtgcatgggggtgggggtggggttagaggggaacagctccagatggcaaacatacgcaagggatttagtcaaacaactttttggcaaagatggtatgattttgtaatggggtaggaaccaatgaaatgcgaggtaagtatggttaataatctacagttattggttaaagaagtatattagagcgagtctttctgcacacagatcaccttcctatcaaccccactagcctctggcaaaggtaccagtgtacagggagtcgctgcgttgccttcgccccgtgccccgctccgcgccgcctcgcgccgcccgccccggctctgactgaccgcgttactcccacaggtgagcgggcgggacggcccttctcctccgggctgtaattagcaagaggtaagggtttaagggatggttggttggtggggtattaatgtttaattacctggagcacctgcctgaaatcactttttttcaggttggacgcgtgccgccaccatgggctggagctgcattattctgtttctggtggcgaccgcgaccggcgtgcatagcgaggtgcagctggtggagagcggcggcggcctggtgcagcccggcaacagcctgaccctgagctgcgtggccagcggcttcaccttcagcaactacggcatgcactggatcaggcaggcccccaagaagggcctggagtggatcgccatgatcgcctacgacagcagcaagatgaactacgccgacaccgtgaagggccgcttcaccatcagccgcgacaacagcaagaacaccctgtacctggagatgaacagcctgcgcagcgaggacaccgccatgtactactgcgccgtgcccaccgcccactacgtggtggacgtgtggggacaaggcgtgagcgtgaccgtgagcagcggtggcggagggtctggcggaggaggttccgggggcggtggaagcgacatccagatgacccagagccccgccagtctgagcgccagcctggaggagatcgtgaccatcacctgccaggcaagccaagacatcggcaactggctggcctggtaccagcagaagcccggcaagagcccccagctgctgatctacggcgccaccagcctggccgacggcgtgcccagccgcttcagcggcagccgcagcggcacccagttcagcctgaagatcagccgcgtgcaggtggaggacatcggcatctactactgcctgcaggcctacaacaccccctggaccttcggcggcggcaccaagctggagctgaagcgcggtggcggagggtctggaggtggcggatcaggcggaggaggatcctccgaaacgcaggccaactcgaccacagatgctctgaacgttcttctcatcatcgtggatgacctgcgcccctccctgggctgttatggggataagctggtgaggtccccaaatattgaccaactggcatcccacagcctcctcttccagaatgcctttgcgcagcaagcagtgtgcgccccgagccgcgtttctttcctcactggcaggagacctgacaccacccgcctgtacgacttcaactcctactggagggtgcacgctggaaacttctccaccatcccccagtacttcaaggagaatggctatgtgaccatgtcggtgggaaaagtctttcaccctgggatatcttctaaccataccgatgattctccgtatagctggtcttttccaccttatcatccttcctctgagaagtatgaaaacactaagacatgtcgagggccagatggagaactccatgccaacctgctttgccctgtggatgtgctggatgttcccgagggcaccttgcctgacaaacagagcactgagcaagccatacagttgttggaaaagatgaaaacgtcagccagtcctttcttcctggccgttgggtatcataagccacacatccccttcagataccccaaggaatttcagaagttgtatcccttggagaacatcaccctggcccccgatcccgaggtccctgatggcctaccccctgtggcctacaacccctggatggacatcaggcaacgggaagacgtccaagccttaaacatcagtgtgccgtatggtccaattcctgtggactttcagcggaaaatccgccagagctactttgcctctgtgtcatatttggatacacaggtcggccgcctcttgagtgctttggacgatcttcagctggccaacagcaccatcattgcatttacctcggatcatgggtgggctctaggtgaacatggagaatgggccaaatacagcaattttgatgttgctacccatgttcccctgatattctatgttcctggaaggacggcttcacttccggaggcaggcgagaagcttttcccttacctcgacccttttgattccgcctcacagttgatggagccaggcaggcaatccatggaccttgtggaacttgtgtctctttttcccacgctggctggacttgcaggactgcaggttccacctcgctgccccgttccttcatttcacgttgagctgtgcagagaaggcaagaaccttctgaagcattttcgattccgtgacttggaagaagatccgtacctccctggtaatccccgtgaactgattgcctatagccagtatccccggccttcagacatccctcagtggaattctgacaagccgagtttaaaagatataaagatcatgggctattccatacgcaccatagactataggtatactgtgtgggttggcttcaatcctgatgaatttctagctaacttttctgacatccatgcaggggaactgtattttgtggattctgacccattgcaggatcacaatatgtataatgattcccaaggtggagaccttttccagttgttgatgccttaataagcggccgcatttaaatctgtgccttctagttgccagccatctgttgtttgcccctcccccgtgccttccttgaccctggaaggtgccactcccactgtcctttcctaataaaatgaggaaattgcatcgcattgtctgagtaggtgtcattctattctggggggtggggtggggcaggacagcaagggggaggattgggaagacaatagcaggcatgctggggaagatct

SEQ ID NO: 58 - protein, 883 aa, Homo sapiens
AHPGRPRAVPTQCDVPPNSRFDCAPDKAITQEQCEARGCCYIPAKQGLQGAQMGQPWCFFPPSYPSYKLENLSSSEMGYTATLTRTTPTFFPKDILTLRLDVMMETENRLHFTIKDPANRRYEVPLETPHVHSRAPSPLYSVEFSEEPFGVIVRRQLDGRVLLNTTVAPLFFADQFLQLSTSLPSQYITGLAEHLSPLMLSTSWTRITLWNRDLAPTPGANLYGSHPFYLALEDGGSAHGVFLLNSNAMDVVLQPSPALSWRSTGGILDVYIFLGPEPKSVVQQYLDVVGYPFMPPYWGLGFHLCRWGYSSTAITRQVVENMTRAHFPLDVQWNDLDYMDSRRDFTFNKDGFRDFPAMVQELHQGGRRYMMIVDPAISSSGPAGSYRPYDEGLRRGVFITNETGQPLIGKVWPGSTAFPDFTNPTALAWWEDMVAEFHDQVPFDGMWIDMNEPSNFIRGSEDGCPNNELENPPYVPGVVGGTLQAATICASSHQFLSTHYNLHNLYGLTEAIASHRALVKARGTRPFVISRSTFAGHGRYAGHWTGDVWSSWEQLASSVPEILQFNLLGVPLVGADVCGFLGNTSEELCVRWTQLGAFYPFMRNHNSLLSLPQEPYSFSEPAQQAMRKALTLRYALLPHLYTLFHQAHVAGETVARPLFLEFPKDSSTWTVDHQLLWGEALLITPVLQAGKAEVTGYFPLGTWYDLQTVPVEALGSLPPPPAAPREPAIHSEGQWVTLPAPLDTINVHLRAGYIIPLQGPGLTTTESRQQPMALAVALTKGGEARGELFWDDGESLEVLERGAYTQVIFLARNNTIVNELVRVTSEGAGLQLQKVTVLGVATAPQQVLSNGVPVSNFTYSPDTKVLDICVSLLMGEQFLVSWC

SEQ ID NO: 59 - DNA, 2669 bp, synthetic construct
  source 1..2669: mol_type = other DNA
ggatccgcccaccctggcagacctagagccgtgcctacacagtgcgacgtgcctcctaacagcagattcgactgcgcccctgacaaggccatcacccaagagcagtgtgaggctagaggctgctgttacatccctgccaagcaaggcctgcaaggcgctcagatgggacagccttggtgcttcttccctcctagctaccctagctacaagctggagaatctgagcagcagcgagatgggctacaccgccaccctgacaagaaccacccctaccttctttcccaaggacatcctcacccttcggctggacgtgatgatggagaccgagaacagactgcacttcaccatcaaggaccctgccaacagaagatacgaggtgcctctggagacccctcacgtgcacagcagagcccctagccctctgtacagcgtggagttcagcgaggagcctttcggcgtgatcgtgagaagacagctggacggcagagtgctgctgaacaccaccgtggcccctctgttcttcgccgatcagttcctgcagctgagtacctcgctcccttctcagtacatcaccggcctggccgagcacctgagccctctgatgctgagcacaagctggacaagaatcaccctgtggaacagagacctggcccctacccctggcgccaatctgtacggttcgcaccctttctacctggccctggaggacggcggcagcgcccacggcgtgttcctgctgaacagcaacgccatggacgtggtgctgcagcctagccctgccctgagctggagaagcaccggcggcatcctggacgtgtacatcttcctgggccctgagcctaagagcgtggtgcagcagtacctggacgtggtgggctatcctttcatgcccccctactggggcctgggcttccacctgtgcagatggggctacagcagcaccgccatcacaagacaagtggtggagaacatgacaagagcccatttccctcttgatgtacagtggaacgacctggactacatggacagcagaagagacttcaccttcaacaaggacggcttcagagacttccctgccatggtgcaagagctgcaccaaggcggcagaagatacatgatgatcgtggaccctgccatcagcagcagcggccctgccggcagctacagaccttacgacgagggcctgagaagaggcgtgttcatcaccaacgagaccggacagcctctgatcggcaaggtgtggcctggcagcaccgccttccctgacttcaccaaccctaccgccctggcctggtgggaggacatggtggccgagttccacgaccaagtgcctttcgacggcatgtggatcgacatgaacgagcctagcaacttcatcagaggcagcgaggacggctgccctaacaatgagttagagaaccctccctacgtgcctggcgttgtcggcggcacgctgcaagccgccaccatctgcgctagcagccatcagttcctgagcacccactacaacctgcacaatctgtatggactgacggaggccatcgctagccacagagccctggtgaaggctagaggcacaagacctttcgtgatcagcagaagcaccttcgccggccacggcagatacgccggccactggaccggcgacgtgtggagcagctgggagcagctggctagcagcgtgcctgagatcctgcagttcaacctgctgggcgtgcctctggtgggcgccgacgtgtgcggcttcctgggcaacacaagcgaggagctgtgcgtgagatggacacagctgggcgccttctaccctttcatgagaaatcacaacagcctgctgagcctgcctcaagagccttacagcttcagcgagcctgctcagcaagccatgagaaaggccctgacccttcgctacgccctgctgcctcacctgtacaccctgttccaccaagcccacgtggccggcgagaccgtggctagacctctgttcctggagttccctaaagacagtagcacctggaccgtggaccatcagctgctgtggggcgaggccctgctgatcacccctgtgctgcaagccggcaaggccgaggtgaccggctatttccctctgggcacctggtacgatctgcagaccgtgcctgtggaagcgctgggcagcctgcctcctcctcctgccgcccctagagagcctgccatccacagcgagggacagtgggtgaccctgcctgcccctctggacaccatcaacgtgcacctgagagccggctacatcatccctctgcaaggccctggcctgaccaccaccgagagcagacagcagcctatggccctggccgtggccctgaccaagggcggcgaagctagaggcgagctcttctgggacgacggcgagtcgctggaggtgctggagagaggcgcctacacccaagtgatcttcctggctagaaacaacaccatcgtgaacgagctggtgagagtgactagcgaaggggccggcctgcagctgcagaaggtgaccgtgctgggcgttgccaccgcccctcagcaagtgctgagcaacggcgtgcctgtgagcaacttcacctacagccctgacaccaaggtgctggacatctgcgtgagcctgctgatgggcgagcagttcctggtgagctggtgctaataagcggccgc

SEQ ID NO: 60 - protein, 1139 aa, synthetic construct
EVQLVESGGGLVQPGNSLTLSCVASGFTFSNYGMHWIRQAPKKGLEWIAMIYYDSSKMNYADTVKGRFTISRDNSKNTLYLEMNSLRSEDTAMYYCAVPTSHYVVDVWGQGVSVTVSSGGGGSGGGGSGGGGSDIQMTQSPASLSASLEEIVTITCQASQDIGNWLAWYQQKPGKSPQLLIYGATSLADGVPSRFSGSRSGTQFSLKISRVQVEDIGIYYCLQAYNTPWTFGGGTKLELKRGGGGSGGGGSGGGGSAHPGRPRAVPTQCDVPPNSRFDCAPDKAITQEQCEARGCCYIPAKQGLQGAQMGQPWCFFPPSYPSYKLENLSSSEMGYTATLTRTTPTFFPKDILTLRLDVMMETENRLHFTIKDPANRRYEVPLETPHVHSRAPSPLYSVEFSEEPFGVIVRRQLDGRVLLNTTVAPLFFADQFLQLSTSLPSQYITGLAEHLSPLMLSTSWTRITLWNRDLAPTPGANLYGSHPFYLALEDGGSAHGVFLLNSNAMDVVLQPSPALSWRSTGGILDVYIFLGPEPKSVVQQYLDVVGYPFMPPYWGLGFHLCRWGYSSTAITRQVVENMTRAHFPLDVQWNDLDYMDSRRDFTFNKDGFRDFPAMVQELHQGGRRYMMIVDPAISSSGPAGSYRPYDEGLRRGVFITNETGQPLIGKVWPGSTAFPDFTNPTALAWWEDMVAEFHDQVPFDGMWIDMNEPSNFIRGSEDGCPNNELENPPYVPGVVGGTLQAATICASSHQFLSTHYNLHNLYGLTEAIASHRALVKARGTRPFVISRSTFAGHGRYAGHWTGDVWSSWEQLASSVPEILQFNLLGVPLVGADVCGFLGNTSEELCVRWTQLGAFYPFMRNHNSLLSLPQEPYSFSEPAQQAMRKALTLRYALLPHLYTLFHQAHVAGETVARPLFLEFPKDSSTWTVDHQLLWGEALLITPVLQAGKAEVTGYFPLGTWYDLQTVPVEALGSLPPPPAAPREPAIHSEGQWVTLPAPLDTINVHLRAGYIIPLQGPGLTTTESRQQPMALAVALTKGGEARGELFWDDGESLEVLERGAYTQVIFLARNNTIVNELVRVTSEGAGLQLQKVTVLGVATAPQQVLSNGVPVSNFTYSPDTKVLDICVSLLMGEQFLVSWC

SEQ ID NO: 61 - protein, 925 aa, Homo sapiens
GHILLHDFLLVPRELSGSSPVLEETHPAHQQGASRPGPRDAQAHPGRPRAVPTQCDVPPNSRFDCAPDKAITQEQCEARGCCYIPAKQGLQGAQMGQPWCFFPPSYPSYKLENLSSSEMGYTATLTRTTPTFFPKDILTLRLDVMMETENRLHFTIKDPANRRYEVPLETPHVHSRAPSPLYSVEFSEEPFGVIVRRQLDGRVLLNTTVAPLFFADQFLQLSTSLPSQYITGLAEHLSPLMLSTSWTRITLWNRDLAPTPGANLYGSHPFYLALEDGGSAHGVFLLNSNAMDVVLQPSPALSWRSTGGILDVYIFLGPEPKSVVQQYLDVVGYPFMPPYWGLGFHLCRWGYSSTAITRQVVENMTRAHFPLDVQWNDLDYMDSRRDFTFNKDGFRDFPAMVQELHQGGRRYMMIVDPAISSSGPAGSYRPYDEGLRRGVFITNETGQPLIGKVWPGSTAFPDFTNPTALAWWEDMVAEFHDQVPFDGMWIDMNEPSNFIRGSEDGCPNNELENPPYVPGVVGGTLQAATICASSHQFLSTHYNLHNLYGLTEAIASHRALVKARGTRPFVISRSTFAGHGRYAGHWTGDVWSSWEQLASSVPEILQFNLLGVPLVGADVCGFLGNTSEELCVRWTQLGAFYPFMRNHNSLLSLPQEPYSFSEPAQQAMRKALTLRYALLPHLYTLFHQAHVAGETVARPLFLEFPKDSSTWTVDHQLLWGEALLITPVLQAGKAEVTGYFPLGTWYDLQTVPVEALGSLPPPPAAPREPAIHSEGQWVTLPAPLDTINVHLRAGYIIPLQGPGLTTTESRQQPMALAVALTKGGEARGELFWDDGESLEVLERGAYTQVIFLARNNTIVNELVRVTSEGAGLQLQKVTVLGVATAPQQVLSNGVPVSNFTYSPDTKVLDICVSLLMGEQFLVSWC

SEQ ID NO: 62 - DNA, 2893 bp, synthetic construct
  source 1..2893: mol_type = other DNA
acgcgtgccgccaccatgggcgtgagacaccctccttgttcgcatcgtttgctggccgtgtgcgccctggtgtcactcgccaccgctgccctgctgggccacatcctgctgcacgacttcctgctggtgcctagagagctgtcgggctcctcgcctgtgttggaggagacccaccctgcacatcagcaaggcgcctctagacctgggcctagagacgcccaagcccaccctggcagacctagagccgtgcctacacagtgcgacgtgcctcctaacagcagattcgactgcgcccctgacaaggccatcacccaagagcagtgtgaggctagaggctgctgttacatccctgccaagcaaggcctgcaaggcgctcagatgggacagccttggtgcttcttccctcctagctaccctagctacaagctggagaatctgagcagcagcgagatgggctacaccgccaccctgacaagaaccacccctaccttctttcccaaggacatcctcacccttcggctggacgtgatgatggagaccgagaacagactgcacttcaccatcaaggaccctgccaacagaagatacgaggtgcctctggagacccctcacgtgcacagcagagcccctagccctctgtacagcgtggagttcagcgaggagcctttcggcgtgatcgtgagaagacagctggacggcagagtgctgctgaacaccaccgtggcccctctgttcttcgccgatcagttcctgcagctgagtacctcgctcccttctcagtacatcaccggcctggccgagcacctgagccctctgatgctgagcacaagctggacaagaatcaccctgtggaacagagacctggcccctacccctggcgccaatctgtacggttcgcaccctttctacctggccctggaggacggcggcagcgcccacggcgtgttcctgctgaacagcaacgccatggacgtggtgctgcagcctagccctgccctgagctggagaagcaccggcggcatcctggacgtgtacatcttcctgggccctgagcctaagagcgtggtgcagcagtacctggacgtggtgggctatcctttcatgcccccctactggggcctgggcttccacctgtgcagatggggctacagcagcaccgccatcacaagacaagtggtggagaacatgacaagagcccatttccctcttgatgtacagtggaacgacctggactacatggacagcagaagagacttcaccttcaacaaggacggcttcagagacttccctgccatggtgcaagagctgcaccaaggcggcagaagatacatgatgatcgtggaccctgccatcagcagcagcggccctgccggcagctacagaccttacgacgagggcctgagaagaggcgtgttcatcaccaacgagaccggacagcctctgatcggcaaggtgtggcctggcagcaccgccttccctgacttcaccaaccctaccgccctggcctggtgggaggacatggtggccgagttccacgaccaagtgcctttcgacggcatgtggatcgacatgaacgagcctagcaacttcatcagaggcagcgaggacggctgccctaacaatgagttagagaaccctccctacgtgcctggcgttgtcggcggcacgctgcaagccgccaccatctgcgctagcagccatcagttcctgagcacccactacaacctgcacaatctgtatggactgacggaggccatcgctagccacagagccctggtgaaggctagaggcacaagacctttcgtgatcagcagaagcaccttcgccggccacggcagatacgccggccactggaccggcgacgtgtggagcagctgggagcagctggctagcagcgtgcctgagatcctgcagttcaacctgctgggcgtgcctctggtgggcgccgacgtgtgcggcttcctgggcaacacaagcgaggagctgtgcgtgagatggacacagctgggcgccttctaccctttcatgagaaatcacaacagcctgctgagcctgcctcaagagccttacagcttcagcgagcctgctcagcaagccatgagaaaggccctgacccttcgctacgccctgctgcctcacctgtacaccctgttccaccaagcccacgtggccggcgagaccgtggctagacctctgttcctggagttccctaaagacagtagcacctggaccgtggaccatcagctgctgtggggcgaggccctgctgatcacccctgtgctgcaagccggcaaggccgaggtgaccggctatttccctctgggcacctggtacgatctgcagaccgtgcctgtggaagcgctgggcagcctgcctcctcctcctgccgcccctagagagcctgccatccacagcgagggacagtgggtgaccctgcctgcccctctggacaccatcaacgtgcacctgagagccggctacatcatccctctgcaaggccctggcctgaccaccaccgagagcagacagcagcctatggccctggccgtggccctgaccaagggcggcgaagctagaggcgagctcttctgggacgacggcgagtcgctggaggtgctggagagaggcgcctacacccaagtgatcttcctggctagaaacaacaccatcgtgaacgagctggtgagagtgactagcgaaggggccggcctgcagctgcagaaggtgaccgtgctgggcgttgccaccgcccctcagcaagtgctgagcaacggcgtgcctgtgagcaacttcacctacagccctgacaccaaggtgctggacatctgcgtgagcctgctgatgggcgagcagttcctggtgagctggtgcggcggcggcggatcccctgagg

SEQ ID NO: 63 - protein, 1171 aa, synthetic construct
GHILLHDFLLVPRELSGSSPVLEETHPAHQQGASRPGPRDAQAHPGRPRAVPTQCDVPPNSRFDCAPDKAITQEQCEARGCCYIPAKQGLQGAQMGQPWCFFPPSYPSYKLENLSSSEMGYTATLTRTTPTFFPKDILTLRLDVMMETENRLHFTIKDPANRRYEVPLETPHVHSRAPSPLYSVEFSEEPFGVIVRRQLDGRVLLNTTVAPLFFADQFLQLSTSLPSQYITGLAEHLSPLMLSTSWTRITLWNRDLAPTPGANLYGSHPFYLALEDGGSAHGVFLLNSNAMDVVLQPSPALSWRSTGGILDVYIFLGPEPKSVVQQYLDVVGYPFMPPYWGLGFHLCRWGYSSTAITRQVVENMTRAHFPLDVQWNDLDYMDSRRDFTFNKDGFRDFPAMVQELHQGGRRYMMIVDPAISSSGPAGSYRPYDEGLRRGVFITNETGQPLIGKVWPGSTAFPDFTNPTALAWWEDMVAEFHDQVPFDGMWIDMNEPSNFIRGSEDGCPNNELENPPYVPGVVGGTLQAATICASSHQFLSTHYNLHNLYGLTEAIASHRALVKARGTRPFVISRSTFAGHGRYAGHWTGDVWSSWEQLASSVPEILQFNLLGVPLVGADVCGFLGNTSEELCVRWTQLGAFYPFMRNHNSLLSLPQEPYSFSEPAQQAMRKALTLRYALLPHLYTLFHQAHVAGETVARPLFLEFPKDSSTWTVDHQLLWGEALLITPVLQAGKAEVTGYFPLGTWYDLQTVPVEALGSLPPPPAAPREPAIHSEGQWVTLPAPLDTINVHLRAGYIIPLQGPGLTTTESRQQPMALAVALTKGGEARGELFWDDGESLEVLERGAYTQVIFLARNNTIVNELVRVTSEGAGLQLQKVTVLGVATAPQQVLSNGVPVSNFTYSPDTKVLDICVSLLMGEQFLVSWCGGGGSEVQLVESGGGLVQPGNSLTLSCVASGFTFSNYGMHWIRQAPKKGLEWIAMIAYDSSKMNYADTVKGRFTISRDNSKNTLYLEMNSLRSEDTAMYYCAVPTAHYVVDVWGQGVSVTVSSGGGGSGGGGSGGGGSDIQMTQSPASLSASLEEIVTITCQASQDIGNWLAWYQQKPGKSPQLLIAGATSLADGVPSRFSGSRSGTQFSLKISRVQVEDIGIYYCLQAANTPWTFGGGTKLELKR

SEQ ID NO: 64 - DNA, 2885 bp, synthetic construct
  source 1..2885: mol_type = other DNA
acgcgtgccgccaccatgggcgtgagacaccctccttgttcgcatcgtttgctggccgtgtgcgccctggtgtcactcgccaccgctgccctgctgggccacatcctgctgcacgacttcctgctggtgcctagagagctgtcgggctcctcgcctgtgttggaggagacccaccctgcacatcagcaaggcgcctctagacctgggcctagagacgcccaagcccaccctggcagacctagagccgtgcctacacagtgcgacgtgcctcctaacagcagattcgactgcgcccctgacaaggccatcacccaagagcagtgtgaggctagaggctgctgttacatccctgccaagcaaggcctgcaaggcgctcagatgggacagccttggtgcttcttccctcctagctaccctagctacaagctggagaatctgagcagcagcgagatgggctacaccgccaccctgacaagaaccacccctaccttctttcccaaggacatcctcacccttcggctggacgtgatgatggagaccgagaacagactgcacttcaccatcaaggaccctgccaacagaagatacgaggtgcctctggagacccctcacgtgcacagcagagcccctagccctctgtacagcgtggagttcagcgaggagcctttcggcgtgatcgtgagaagacagctggacggcagagtgctgctgaacaccaccgtggcccctctgttcttcgccgatcagttcctgcagctgagtacctcgctcccttctcagtacatcaccggcctggccgagcacctgagccctctgatgctgagcacaagctggacaagaatcaccctgtggaacagagacctggcccctacccctggcgccaatctgtacggttcgcaccctttctacctggccctggaggacggcggcagcgcccacggcgtgttcctgctgaacagcaacgccatggacgtggtgctgcagcctagccctgccctgagctggagaagcaccggcggcatcctggacgtgtacatcttcctgggccctgagcctaagagcgtggtgcagcagtacctggacgtggtgggctatcctttcatgcccccctactggggcctgggcttccacctgtgcagatggggctacagcagcaccgccatcacaagacaagtggtggagaacatgacaagagcccatttccctcttgatgtacagtggaacgacctggactacatggacagcagaagagacttcaccttcaacaaggacggcttcagagacttccctgccatggtgcaagagctgcaccaaggcggcagaagatacatgatgatcgtggaccctgccatcagcagcagcggccctgccggcagctacagaccttacgacgagggcctgagaagaggcgtgttcatcaccaacgagaccggacagcctctgatcggcaaggtgtggcctggcagcaccgccttccctgacttcaccaaccctaccgccctggcctggtgggaggacatggtggccgagttccacgaccaagtgcctttcgacggcatgtggatcgacatgaacgagcctagcaacttcatcagaggcagcgaggacggctgccctaacaatgagttagagaaccctccctacgtgcctggcgttgtcggcggcacgctgcaagccgccaccatctgcgctagcagccatcagttcctgagcacccactacaacctgcacaatctgtatggactgacggaggccatcgctagccacagagccctggtgaaggctagaggcacaagacctttcgtgatcagcagaagcaccttcgccggccacggcagatacgccggccactggaccggcgacgtgtggagcagctgggagcagctggctagcagcgtgcctgagatcctgcagttcaacctgctgggcgtgcctctggtgggcgccgacgtgtgcggcttcctgggcaacacaagcgaggagctgtgcgtgagatggacacagctgggcgccttctaccctttcatgagaaatcacaacagcctgctgagcctgcctcaagagccttacagcttcagcgagcctgctcagcaagccatgagaaaggccctgacccttcgctacgccctgctgcctcacctgtacaccctgttccaccaagcccacgtggccggcgagaccgtggctagacctctgttcctggagttccctaaagacagtagcacctggaccgtggaccatcagctgctgtggggcgaggccctgctgatcacccctgtgctgcaagccggcaaggccgaggtgaccggctatttccctctgggcacctggtacgatctgcagaccgtgcctgtggaagcgctgggcagcctgcctcctcctcctgccgcccctagagagcctgccatccacagcgagggacagtgggtgaccctgcctgcccctctggacaccatcaacgtgcacctgagagccggctacatcatccctctgcaaggccctggcctgaccaccaccgagagcagacagcagcctatggccctggccgtggccctgaccaagggcggcgaagctagaggcgagctcttctgggacgacggcgagtcgctggaggtgctggagagaggcgcctacacccaagtgatcttcctggctagaaacaacaccatcgtgaacgagctggtgagagtgactagcgaaggggccggcctgcagctgcagaaggtgaccgtgctgggcgttgccaccgcccctcagcaagtgctgagcaacggcgtgcctgtgagcaacttcacctacagccctgacaccaaggtgctggacatctgcgtgagcctgctgatgggcgagcagttcctggtgagctggtgctaataagcggccgc